European Patent Application EP 4 198 133 A1, published June 21, 2023. Title: GLYCOALKALOID METABOLISM ENYZYMES (GAMES) AND USES THEREOF. Applicant: YEDA RESEARCH AND DEVELOPMENT CO. LTD. Application IL PCT/IL2018/050142, filed February 8, 2018. The sequence listing filed with the application follows.

SEQUENCE LISTING (107 sequences)

SEQ ID NO: 1 - DNA, 1468 bp, Solanum lycopersicum
  source 1..1468: mol_type = other DNA
gtgatatatttcaaaaaataattaaaatacatatatattgcatacataattcacttttaatacatattgcagatttaacttaaacattgttataaatggtgataaataaaaaaatcgttaaaattagtaattattcattaaactgcatctatttatgtaatttttccaattaaaaatctattattttttttcaatccaatccaaacaggctctaaagcatcaatgtttttgaaattaccaaaatagcctcggttgttaagcgcttccttctatatattagtgaattcaaactacagtcggtacaaaggaagttatttactcttataatggcaaataagctcaggtatagcatagttagtatttgtttaaattaatggtgctaatcagtacattaatttattttctcaaaattgtgtaattacatataattaaatgtgtttaatcaaatgtttttcttttttatatgcatcgatcctgtaggttggagggcaaagtagctataattaccggtgctgctagtggcattggagaagcaagtgctagattgttcgttgaacatggtgctcgtgtcgtcgtcgccgatattcaagatgaacttggtcaaaaagtagttgattctatcggatctgacaaagccagctaccggcactgcgacgttacagacgagaagcaagttgaggaaaccgtagcttacgcggtagagaaatacggtactcttgacattatgtttagtaatgtcgggacgctgaatttctgcagcgtcctcgacatggacgtgctggccttcgatgagaccatggccatcaacgtacgcggatccgcgttagcggttaagcacgcggctaaagttatggttgataagaaaattcggggatctattatatgtaacgcgagtttagaagggattttagctggggccgcttcgctcgcctacattgcgtcaaagcacgcagtggtaggcattataaaagcggccgcacgtgaactgggtccacatgggataagggtgaatggggtgtcgccctatggaatagcgacgccccttgtgactaaggcgtatggactggatgcggctctattggaagaagcaatttacggtaatggacacttgaaaggagttaagttgagcacgatgcatgtagcacaatcagcactttttttggcgtctgatgaatctgcttatacaagtggtcaaaatttagctgttgatggtggactaagttctattttgaagctacaataaattgtcacgctatttgtgttggcgtgctgtggcgtgggccttaatcctcactctcttgtgtctgtacttctgtttcatctcgtttcgtttcaaattttcaacttaataatactctcatattttatgcgatatttttcagatttatactaagttttttatagatattttaaacgttgtgacttaaaaagatataaatttcatttttttaaaattaaaaattttatg

SEQ ID NO: 2 - DNA, 780 bp, synthetic construct
  misc_feature 1..780: note = GAME25 CDS of Solanum Lycopersicum
  source 1..780: mol_type = other DNA
atggcaaataagctcaggttggagggcaaagtagctataattaccggtgctgctagtggcattggagaagcaagtgctagattgttcgttgaacatggtgctcgtgtcgtcgtcgccgatattcaagatgaacttggtcaaaaagtagttgattctatcggatctgacaaagccagctaccggcactgcgacgttacagacgagaagcaagttgaggaaaccgtagcttacgcggtagagaaatacggtactcttgacattatgtttagtaatgtcgggacgctgaatttctgcagcgtcctcgacatggacgtgctggccttcgatgagaccatggccatcaacgtacgcggatccgcgttagcggttaagcacgcggctaaagttatggttgataagaaaattcggggatctattatatgtaacgcgagtttagaagggattttagctggggccgcttcgctcgcctacattgcgtcaaagcacgcagtggtaggcattataaaagcggccgcacgtgaactgggtccacatgggataagggtgaatggggtgtcgccctatggaatagcgacgccccttgtgactaaggcgtatggactggatgcggctctattggaagaagcaatttacggtaatggacacttgaaaggagttaagttgagcacgatgcatgtagcacaatcagcactttttttggcgtctgatgaatctgcttatacaagtggtcaaaatttagctgttgatggtggactaagttctattttgaagctacaataa

SEQ ID NO: 3 - protein, 259 aa, Solanum lycopersicum
MANKLRLEGKVAIITGAASGIGEASARLFVEHGARVVVADIQDELGQKVVDSIGSDKASYRHCDVTDEKQVEETVAYAVEKYGTLDIMFSNVGTLNFCSVLDMDVLAFDETMAINVRGSALAVKHAAKVMVDKKIRGSIICNASLEGILAGAASLAYIASKHAVVGIIKAAARELGPHGIRVNGVSPYGIATPLVTKAYGLDAALLEEAIYGNGHLKGVKLSTMHVAQSALFLASDESAYTSGQNLAVDGGLSSILKLQ

SEQ ID NO: 4 - DNA, 24 bp, synthetic construct
  misc_feature 1..24: note = GAME25 qRT Forward primer
  source 1..24: mol_type = other DNA
gaagcaatttacggtaatggacac

SEQ ID NO: 5 - DNA, 23 bp, synthetic construct
  misc_feature 1..23: note = GAME25 qRT Reverse primer
  source 1..23: mol_type = other DNA
gaacttagtccaccatcaacagc

SEQ ID NO: 6 - DNA, 30 bp, synthetic construct
  misc_feature 1..30: note = GAME25 RNAi Forward primer
  source 1..30: mol_type = other DNA
gcggccgcattgtcacgctatttgtgttgg

SEQ ID NO: 7 - DNA, 36 bp, synthetic construct
  misc_feature 1..36: note = GAME25 RNAi Reverse primer
  source 1..36: mol_type = other DNA
ggcgcgccgaaatttatatctttttaagtcacaacg

SEQ ID NO: 8 - DNA, 199 bp, synthetic construct
  misc_feature 1..199: note = GAME25-RNAi construct
  source 1..199: mol_type = other DNA
attgtcacgctatttgtgttggcgtgctgtggcgtgggccttaatcctcactctcttgtgtctgtacttctgtttcatctcgtttcgtttcaaattttcaacttaataatactctcatattttatgcgatatttttcagatttatactaagttttttatagatattttaaacgttgtgacttaaaaagatataaatttc

SEQ ID NO: 9 - DNA, 28 bp, synthetic construct
  misc_feature 1..28: note = GAME25 baculo Forward primer
  source 1..28: mol_type = other DNA
cccgggatggcaaataagctcaggttgg

SEQ ID NO: 10 - DNA, 66 bp, synthetic construct
  misc_feature 1..66: note = GAME25 baculo Reverese primer
  source 1..66: mol_type = other DNA
tctagattacagatcttcttcagaaataagtttttgttcttgtagcttcaaaatagaacttagtcc

SEQ ID NO: 11 - DNA, 780 bp, synthetic construct
  misc_feature 1..780: note = GAME25 CDS of Solanum pennellii
  source 1..780: mol_type = other DNA
atggcaaataagctcaggttggagggcaaagtagctataattactggtgctgctagtggcattggagaggcaagtgctagattgttcgttgaacatggtgctcgtgtcgtcgtcgccgatattcaagatgaacttggtcaaaaagtagttgattctatcggagctgacaaagccagctaccggcactgcgacgttacagacgagaagcaagttgaggaaaccgtagcctacgcggtagagaaatacggtactcttgacattatgtttagtaatgtcgggacgctgaatttctgcagcgtcctcgacatggacgtgatggccttcgatgagacgatggccatcaacgtacgtggatccgcgctagcggttaagcacgcggctaaagttatggttgataagaaaattcggggatctattatatgtaacgcgagtttagaggggattttagctggggccgcttcgcttgcctacattgcgtcaaagcacgcagtcgtaggcataataaaagcggccgcacgtgaactgggtccacatgggataagggtgaatggggtgtcgccatatggaatagcgacgcccctggtgtgtaaggcgtatggactggatgcggctctattggaagaagcaatttatggtaatggacacttgaaaggtgttaagttgagcacgatgcatgtagcacaatcagcactttttttggcgtctgatgaatctgcttacacaagtggtcaaaatttagctgttgatggtggactaagttctattttgaagctacaataa

SEQ ID NO: 12 - protein, 259 aa, Solanum pennellii
MANKLRLEGKVAIITGAASGIGEASARLFVEHGARVVVADIQDELGQKVVDSIGADKASYRHCDVTDEKQVEETVAYAVEKYGTLDIMFSNVGTLNFCSVLDMDVMAFDETMAINVRGSALAVKHAAKVMVDKKIRGSIICNASLEGILAGAASLAYIASKHAVVGIIKAAARELGPHGIRVNGVSPYGIATPLVCKAYGLDAALLEEAIYGNGHLKGVKLSTMHVAQSALFLASDESAYTSGQNLAVDGGLSSILKLQ

SEQ ID NO: 13 - DNA, 1080 bp, Solanum tubersoum
  source 1..1080: mol_type = other DNA
aaaaaatttaacatacagttgctgcaaaggaagctacctactcgtataatggcaaataagctcaggtacttaattagtacattaatttctttctttcttttctcaaattgtatatgagaattaaatgtgtatttttagctttaatcaaatgtttttgtggtatattatatgcatcgtgtaggttggagggcaaagtggctataattacaggtgctgcaagtggcattggagaagcaagtgctagattgttcgccgaacatggtgctcgtattgtcgtagccgatattcaagatgaacttggtctgaaagtagttgaatctatcggagctgacaaagccagctaccgacactgcgacgttacagacgagaagcaagttgaggataccgtagcttacacggtagagaaatacggtactcttgacatcatgtttagtaatgttgggacgctgaatttttgcagcgtcctggacatggacgtgatggtcttcgataagacgatggccatcaacgcacgaggatccgcgttagcggtcaagcacgcggctagatttatggttgataagaaaattcggggatccattatatgcaacgcgagtttagatggtattgtagctggggccacttcgcttgcctacattgcgtcaaagcacgcagttgtaggcattgtgaaagcggccgcacgtgacctaggtccatacgggataagggtgaatggggtgtcgccatatggaatagcgacgcccctggtgtgcaaagcgtatgggttggatgcgggtccattggaagcagcaatatatggaaatggaaacttgaaaggtgttaggttgagcacgatgcatgtagcacaatcagcacttttcttggcgtctgatgaatctgcttacacaagtggtcaaaatttagctgttgatggtggacttagttctattttgaaggtacaatagattgtcactctattgtgctggtgtgctgtgatgtgtgcattagttctattttgaagctacaataattcctttgtcatgtagtactgtttatcttgtttcatttcgaattttcaacttaaataatattctctcacag

SEQ ID NO: 14 - DNA, 780 bp, synthetic construct
  misc_feature 1..780: note = CDS of GAME25 of Solanum tubersoum
  source 1..780: mol_type = other DNA
atggcaaataagctcaggttggagggcaaagtggctataattacaggtgctgcaagtggcattggagaagcaagtgctagattgttcgccgaacatggtgctcgtattgtcgtagccgatattcaagatgaacttggtctgaaagtagttgaatctatcggagctgacaaagccagctaccgacactgcgacgttacagacgagaagcaagttgaggataccgtagcttacacggtagagaaatacggtactcttgacatcatgtttagtaatgttgggacgctgaatttttgcagcgtcctggacatggacgtgatggtcttcgataagacgatggccatcaacgcacgaggatccgcgttagcggtcaagcacgcggctagatttatggttgataagaaaattcggggatccattatatgcaacgcgagtttagatggtattgtagctggggccacttcgcttgcctacattgcgtcaaagcacgcagttgtaggcattgtgaaagcggccgcacgtgacctaggtccatacgggataagggtgaatggggtgtcgccatatggaatagcgacgcccctggtgtgcaaagcgtatgggttggatgcgggtccattggaagcagcaatatatggaaatggaaacttgaaaggtgttaggttgagcacgatgcatgtagcacaatcagcacttttcttggcgtctgatgaatctgcttacacaagtggtcaaaatttagctgttgatggtggacttagttctattttgaaggtacaatag

SEQ ID NO: 15 - protein, 259 aa, Solanum tubersoum
MANKLRLEGKVAIITGAASGIGEASARLFAEHGARIVVADIQDELGLKVVESIGADKASYRHCDVTDEKQVEDTVAYTVEKYGTLDIMFSNVGTLNFCSVLDMDVMVFDKTMAINARGSALAVKHAARFMVDKKIRGSIICNASLDGIVAGATSLAYIASKHAVVGIVKAAARDLGPYGIRVNGVSPYGIATPLVCKAYGLDAGPLEAAIYGNGNLKGVRLSTMHVAQSALFLASDESAYTSGQNLAVDGGLSSILKVQ

SEQ ID NO: 16 - DNA, 2552 bp, Solanum lycopersycum
  source 1..2552: mol_type = other DNA
tgactataattgatactcaatctgttgaaatataatgaaccaattcttatcaaaacacagtggagtacaagtaatcacgttggttcctatgaaatggttcatctatttcccattatatataggctacttatttcctcacctataaagtaaaaaactttctagtgttttcttctttcttttgtttttttctctttgctcatattctaaaaatatttcatcaatggcatctatcaaatcagttaaagttcctactatagatttttccaattatcaagagctaaaaccaaacactccactatgggaatccacaaaaattcaagtttttgaagctttacaagaatatggttgttttgaagcaatatatgataaagtttcaaaggaaattagagaggaaacatttgatatgtcaaaagaaatatttgaatttcctttagagactaaagtgaaaaatatctcagaaaaaccaatgcatggctatatggggatgattccacaattgccattgtatgagagtttgtgtattcctgatttgcttaatcctcaaagtcttgaaaaattttctaatatcttttggcctcagggtaatcaacatttctggtatgtttacttttatttctttttcatttttgttttcttattatctttaaattttgttctagtggaactgttcaaaagctactatctttagaaataataatttttattagcttagttgattgattatgcgatattattaatagcttaaaaaaataatttttattagcttagaaataataatttttattaacttagttgattgactatgcgatattattaatagcttaaaagagcttagttgatcagactacgaaagtaaaataaaaagagacggaagtctgtgtctcgcatctattttttattgcaccgtttaaactaaataaaatatagacaacaacatcaaaatatttggtaggaagacacgatttattcaacagaaatatagacaacaacattaaagtatttggtacatgaaatcactatccaataagtgacagttcgttggccttctcattttttataaaataaatagaaacacaagagttgtctcaagtgaaaaaattgaattatgttcaaccttcttcatatgtttatactaatattacatgagcgttaatttttgcagcaatttgataaaatcttattctaatccacttgtggaattggatgggatgttgaaaaggatgatttcggagaatttgggattgaaaaatcacattgatgaattattgaatgccaattacttcctatttagatttacacattataagggatcatcaattgctagtggagatgaaaataataaagctgctggattgggtggccacacggatggtaacttcttgacttttatatcgcaaaatcaagttaatggattgcaaatcaacaaaaatggagaatggattgatgtgattatttcaccaaattcttacgttgttttggccggtgattccttcaaagtaagtattttaagttttgaactagtgttacttatcttgttgggaactgttttgtttgatttttaaaagaaaaaatattaaatgatcaaaaaaattataatatcttttttgttttaaggttaaataaattgatttaaaaatttcatttttaattaaaagagggtagtaaaatgcttaaaaagctaaaataatttagtgtgaaatatattattttattatcattctaatcaaaatttctggtcacaccttatagcataggggtttcagagggccccgagatattttgttttgatcttatatttctcgaatctatgaaaatgttattccactagtgtttatattattttctgaaatgcatatttttgaatgatttgatatatgctcaatattttcatgcaaaactgaaaatgaattttggtattattgaccgtatttgtattgttttactctccaaaaatattatcgatcgcatctatctttgtatttatacaggcttggacaaatggtcgattgcattcacctctccacagagtaacaatgtccggacaaaatgatagactctccattcaattgttttcattatcaaagccaggtcacttcatccaggcaccaaaagaactagtagatgaagaacacccattactcttcaagccatttgaaattcttgaattattcaagtatggtaccacagaagctggctatacagctcctccaagtgatcttttcaagatttattgtggtgtttgatatgctaattgttgaatttccgcttcaacaagcaacttttctaatgagtttcatcttgtttttttaagtagtatgcattttatgtttgaattgttgcagttggcaattcatgtttaatttgtttttgtttttttgagaaaatatttccaatgggtttcgttggaaattcgtcttgtttttttttttcaagtagtgtacatcttatttttggattgttgatgttgagcgctaatgtttaatttgtttgtgttttgaagaggatgattatactctttaagaggattcaccgtaatcttttagtattatttg

SEQ ID NO: 17 - DNA, 1495 bp, synthetic construct
  misc_feature 1..1495: note = cDNA of GAME31 of Solanum lycopersycum
  source 1..1495: mol_type = other DNA
tgactataattgatactcaatctgttgaaatataatgaaccaattcttatcaaaacacagtggagtacaagtaatcacgttggttcctatgaaatggttcatctatttcccattatatataggctacttatttcctcacctataaagtaaaaaactttctagtgttttcttctttcttttgtttttttctctttgctcatattctaaaaatatttcatcaatggcatctatcaaatcagttaaagttcctactatagatttttccaattatcaagagctaaaaccaaacactccactatgggaatccacaaaaattcaagtttttgaagctttacaagaatatggttgttttgaagcaatatatgataaagtttcaaaggaaattagagaggaaacatttgatatgtcaaaagaaatatttgaatttcctttagagactaaagtgaaaaatatctcagaaaaaccaatgcatggctatatggggatgattccacaattgccattgtatgagagtttgtgtattcctgatttgcttaatcctcaaagtcttgaaaaattttctaatatcttttggcctcagggtaatcaacatttctgcaatttgataaaatcttattctaatccacttgtggaattggatgggatgttgaaaaggatgatttcggagaatttgggattgaaaaatcacattgatgaattattgaatgccaattacttcctatttagatttacacattataagggatcatcaattgctagtggagatgaaaataataaagctgctggattgggtggccacacggatggtaacttcttgacttttatatcgcaaaatcaagttaatggattgcaaatcaacaaaaatggagaatggattgatgtgattatttcaccaaattcttacgttgttttggccggtgattccttcaaagcttggacaaatggtcgattgcattcacctctccacagagtaacaatgtccggacaaaatgatagactctccattcaattgttttcattatcaaagccaggtcacttcatccaggcaccaaaagaactagtagatgaagaacacccattactcttcaagccatttgaaattcttgaattattcaagtatggtaccacagaagctggctatacagctcctccaagtgatcttttcaagatttattgtggtgtttgatatgctaattgttgaatttccgcttcaacaagcaacttttctaatgagtttcatcttgtttttttaagtagtatgcattttatgtttgaattgttgcagttggcaattcatgtttaatttgtttttgtttttttgagaaaatatttccaatgggtttcgttggaaattcgtcttgtttttttttttcaagtagtgtacatcttatttttggattgttgatgttgagcgctaatgtttaatttgtttgtgttttgaagaggatgattatactctttaagaggattcaccgtaatcttttagtattatttg

SEQ ID NO: 18 - protein, 321 aa, Solanum lycopersycum
MASIKSVKVPTIDFSNYQELKPNTPLWESTKIQVFEALQEYGCFEAIYDKVSKEIREETFDMSKEIFEFPLETKVKNISEKPMHGYMGMIPQLPLYESLCIPDLLNPQSLEKFSNIFWPQGNQHFCNLIKSYSNPLVELDGMLKRMISENLGLKNHIDELLNANYFLFRFTHYKGSSIASGDENNKAAGLGGHTDGNFLTFISQNQVNGLQINKNGEWIDVIISPNSYVVLAGDSFKAWTNGRLHSPLHRVTMSGQNDRLSIQLFSLSKPGHFIQAPKELVDEEHPLLFKPFEILELFKYGTTEAGYTAPPSDLFKIYCGV

SEQ ID NO: 19 - DNA, 462 bp, Solanum lycoperscum
  source 1..462: mol_type = other DNA
atggcatctaccaaattagttaaagttcccacaatagatttttcaaatcatcaagatctaaaaccaaacactccactatgggaatccaaaaaaattcaagtttttgaagctttgcaagaatatggttgttttgaagcaatttatgataaagttccaaaagatattagagaggaaacatttagtatttcaaaagaaatatttgaatttcctttagagactaaattgaaaaatatttcagaaaaaccaacgcatggatatatgggaatgattccacaattgccattgtatgagagtttgtgtattcctgatttgcttaatcctaaaagtcttcaaagttttgctaatatcttttggcctcagggtaaccaacatttctggtatgtttacttatgtttttatttcgccctagcagaagtgttcaaaagtacgacattagaaattcttagtgacttaattgattga

SEQ ID NO: 20 - DNA, 462 bp, synthetic construct; identical to SEQ ID NO: 19
  misc_feature 1..462: note = cDNA of GAME31-like 1 of Solanum lycopersycum
  source 1..462: mol_type = other DNA

SEQ ID NO: 21 - protein, 153 aa, Solanum lycopersycum
MASTKLVKVPTIDFSNHQDLKPNTPLWESKKIQVFEALQEYGCFEAIYDKVPKDIREETFSISKEIFEFPLETKLKNISEKPTHGYMGMIPQLPLYESLCIPDLLNPKSLQSFANIFWPQGNQHFWYVYLCFYFALAEVFKSTTLEILSDLID

SEQ ID NO: 22 - DNA, 1113 bp, Solanum lycopersycum
  source 1..1113: mol_type = other DNA
tgagatgttgaaaaggatgatttcggagaatttgggattaaaaaatcacattgatgaattattgaatgccaattacatcctatttagatttacacagtataagggatcatcaattgctagtggagatgaaaataataaagcagctggattgggtggccacacagatggtaacttcttgtctattatatcacaaaatgaagttaatggattgcaaatcaacaaaaatggagagtggattgatgtcaacatttcgccaaattcttatgttgttttatccggtgattccttcacagtaagtgttaagttttgagctagtgttattatcttgttgggaactgtgttgtttgattttctaaagggataatgctaaatgacaagaaactcaaaaaatcaataagatatttgttgaatcttacgtctctaaatatattatcatgctagtgttaattatttcccgaaatgcatatttttgaagaatctgacatactgagtgatattctggaagagtccaaccaagacactttgttgaaactacatgctcaatattttcatgcaaaactgaaaatgaatcttgatatttgttgaccctatgttgctctattctccaaaaatactactgcgactatctttgtatttatgcaggcatggacaaatggccgattgcattctcctgttcatagagttgaaatgcccagaggaagtgatagatattccattcaattattttcattatcaaaaccaggtcacttcatcgaggcaccaaaagaaatggtggatgaagaacaccctttgcttttcaagccatttgaaattcttggattacttgggtatggtgccacagaagctggctatacaactcctcccagtgatcttttcaaggcatattgcggtgtctgatatgctaattgcgaatttccatttctattagaataaagttagtatttatgagatttttgttggtaattcatgtttaattggtttgtgtttttttggaaaatatttctaatgtgttccgttggaaattcgtgtgcatcttatgtttggattgttggtattgggaattcatgtttaatttgtttgtgttcttgggcaaataataaatttgaagcggat

SEQ ID NO: 23 - DNA, 547 bp, synthetic construct
  misc_feature 1..547: note = cDNA of GAME31-like 2 of Solanum lycopersycum
  source 1..547: mol_type = other DNA
tgagatgttgaaaaggatgatttcggagaatttgggattaaaaaatcacattgatgaattattgaatgccaattacatcctatttagatttacacagtataagggatcatcaattgctagtggagatgaaaataataaagcagctggattgggtggccacacagatggtaacttcttgtctattatatcacaaaatgaagttaatggattgcaaatcaacaaaaatggagagtggattgatgtcaacatttcgccaaattcttatgttgttttatccggtgattccttcacagcatggacaaatggccgattgcattctcctgttcatagagttgaaatgcccagaggaagtgatagatattccattcaattattttcattatcaaaaccaggtcacttcatcgaggcaccaaaagaaatggtggatgaagaacaccctttgcttttcaagccatttgaaattcttggattacttgggtatggtgccacagaagctggctatacaactcctcccagtgatcttttcaaggcatattgcggtgtctga

SEQ ID NO: 24 - protein, 181 aa, Solanum lycopersycum
EMLKRMISENLGLKNHIDELLNANYILFRFTQYKGSSIASGDENNKAAGLGGHTDGNFLSIISQNEVNGLQINKNGEWIDVNISPNSYVVLSGDSFTAWTNGRLHSPVHRVEMPRGSDRYSIQLFSLSKPGHFIEAPKEMVDEEHPLLFKPFEILGLLGYGATEAGYTTPPSDLFKAYCGV

SEQ ID NO: 25 - DNA, 4148 bp, Solanum lycopersycum
  source 1..4148: mol_type = other DNA
tgactagaaatagacataaaaccctgtactttttgacacacatgtaatagcactttctctatctaatacgcaactctttattaattttgcgtaaattttgagctatttcccattatatataggctacttatttcctcacctcttaagtaaaaaactttcaagtgtttcttctttcttttatttctctttgttcacatattctaaaaatatttcatcaatggcatctatcaaatcagttaaagttcctactatagatttttccaattatcaagagctaaaaccaaacactccactatgggaatccacaaaaattcaagtttttgaagcttttcaagaatatggttgttttgaagcaatatatgataaagttccaaatgaaattagagaggaaacatttgatatgtcaaaagaaatatttgaatttcctttagatactaaagtgaaaaatatttcagaaaaaccaatgcatggatatatgggaatgattccacaattgccattgtatgagagtttgtgtattcctgatttgcttaatcctcaaagtcttcaaaattttgctaatatcttttggcctcagggtaatcaacatttctggtatgtctatttcactgttttcatcttttttattttcttactatcattatctttaaatttaagaaaaaacgataaatatatccttaaatataaatggtatgcagatattctccatcatatttttgggacatatatttttaccgttcaaaaattaaagcatatataccattttatactaatggatatagacgtgtcataatcttatctaccgccccaacattggatcgatggataagattgtgccaagtttcctaatttaaccattcgttagagtgaagggcagaaattttcgactttttaaatgtcagggacatcaatgtcccaaaagtatgacggaggaaaaatataacgaaaaatatgtgcatactatttacgatcgtttgaaaaaatatttgtcttttttccttttaaattttggcctaatgaaagtgttcaaaaagtataacattagagattcccagtaaattgattaactatttgaccattcaatagttttatggaataagttaattttttctttgagaaaaacaaaataggagattataaatggaagtttccttctcgaatctattcattagcacacccctaaacaaacaaaagtgccgataacgttaaaatatttggtatgaagtctcgatctactcaataaaaacaaataaattaataggagacaatagacagtatctttctcgaatcaatttcgaatttatttcttttatcacattgttaataaaatgaaaattatcaacaacatcagaatatttggtatgtgtcacgatctaataattgtagaaatcgagatataaatacgatttgagaaatcaaagattgtattgatgaaaaataatgttaagttacaaggtttttatatggagagaattgtagagttctaagttaactataataaaatactattacaatacatattactattataataataataataatgcaaatcctagtcgtaatataattctaatcgacttcaactagtacaataagtaaataagtagcactgcgtctaatcctagtatgaatctaactcgtcagtcagttccgctttcccatttttgttttcactatcctagttttaaaaataaaataaaatataagacttagttaacgtaaatatggcctcatttgtttgtatttaattgggggtctaaatcttaatcaatcagattcgcctcattcagtatgtttgtttttttatgactgaatcttaattatttagatttaattcattaagtttgtttgttttattttcttagaagtctcttaacgagtctgaatacatctgagttaatcagatctgtaatacactcttaagaccattcagactcaaaagtaattcctatcttaattcaactacatcacaaaaactcataaaagtttttttcttattaaattaatgttaattacatgcttacccgttataatttcctttattttactaacttaatatacgtcctttactttcataaattaatcaatatatttgaattgataaacacttcatgatataatatttagcacgattctagaaaacaagaaagtattgattagttgatcgataacaataacaaatctgcattataaaataaaatgctttcataaacattatattactactctatataaactattttacattgcattatattagattatcaaagtttttgagtgcaaaaaagaatagtcatatattagtgatgtaacttaatgttaaattcttaatagataaatcatatgacctattcatgataagaatgtccaaaaatttattttccatataaaaaattattttactaaaatgaggtttttataattttttgttgatacatcgtttaatttcatatgtacattcaaatattaaaaacgaattatctcaataatccagttttcatattcagagaaaataccttaatattaaaatgtttattcagatttacatatctagatcttaatgcatattttaatatttagatgtatattcagattcagacgttttgatcttaatagaaacaaataaggcctaagtgaaagaatggtatcaacttgaaatgtttctaaatctgttcaaccttctttatatgtttataaacattatatgtgtattttttttttgcagcaatttggtaaagtcttattctaatccacttgtggaattggatgagattttgaaaaggatgatttcggagaatttgagattaaaaattcacattgatgaattgttgaatgccaattatttcctatttagatttacacattacaagggatcatcaattactggtggagatgagaataacaaagttgctggattgggtggccacacagatggtaacttcttgacttttatatcgcaaaatcaagtcaatggattgcaaatcaacaaaaatggagaatggattgatgtgaatatttcaccaaattcttatgttgttttggctggtgattccttcaaagtaagtgttaagttttgaattattgttattatcttgttgggaactgttttgtttgatttttaaaagaaaaatgctaaatggtcacaaatttttaaagtcaataatattttttttgttttaaggtaaataaattgataaaaaaagaattcatttttaattaaaagatattgaaattaaaagggtaaaaatactttaaacatagtgtgaattatgttattttatcattctaatcaaaatttgtggccaatattgttacaccttataggatttatcaaaaaaacatagttttcagaggctcaagatatttgttggatcttatgtttctcgaatctctgaaaatgttgttccgcttgtgttgaatgtattattttctgaaatgtatatttttgaagaatttgatatattaatgatatgctcaatattttcatgcaaaacggaaaatgaattttggtattattgaccctatttgtattgttctactctccaaaaatattatcgatcacgtctatctttgtatttatacaggcttggacaaatggtcgattgcattctcctcttcacagagtaacaatgtccggagaaaatgatagactctccattcaattattttcattatcaaaaccaggtcacttcatcgaggcaccaaaagaactagtggatgaagaacaccctttactcttcaagccatttgaaattattggattatttgagtatggtaccacagaagctggctatacagctcctccaagtgatcttctcaagagttattgcggtgtttgatatgctaattgcgaatttccgcttcagcaaccaacttttctaataagtttcgtctgaaattcgtgttgttttaattattatgcattttatgtttgaattgttgtagttggcaattcatgtttaatttgtttgtgtttttttttttgagaaaatattgcattgggtttcattggaaatttgtgttttttaaaaagtagtgtgcatcttatgtttggattgttggtgttgagaattcatttttaatttgtttttttttttgggcaaataatgaatttaaaattgttgattttactctttagtggaaatgat

SEQ ID NO: 26 - DNA, 1345 bp, synthetic construct
  misc_feature 1..1345: note = cDNA of GAME31-like 3 of Solanum lycopersycum
  source 1..1345: mol_type = other DNA
tgactagaaatagacataaaaccctgtactttttgacacacatgtaatagcactttctctatctaatacgcaactctttattaattttgcgtaaattttgagctatttcccattatatataggctacttatttcctcacctcttaagtaaaaaactttcaagtgtttcttctttcttttatttctctttgttcacatattctaaaaatatttcatcaatggcatctatcaaatcagttaaagttcctactatagatttttccaattatcaagagctaaaaccaaacactccactatgggaatccacaaaaattcaagtttttgaagcttttcaagaatatggttgttttgaagcaatatatgataaagttccaaatgaaattagagaggaaacatttgatatgtcaaaagaaatatttgaatttcctttagatactaaagtgaaaaatatttcagaaaaaccaatgcatggatatatgggaatgattccacaattgccattgtatgagagtttgtgtattcctgatttgcttaatcctcaaagtcttcaaaattttgctaatatcttttggcctcagggtaatcaacatttctgcaatttggtaaagtcttattctaatccacttgtggaattggatgagattttgaaaaggatgatttcggagaatttgagattaaaaattcacattgatgaattgttgaatgccaattatttcctatttagatttacacattacaagggatcatcaattactggtggagatgagaataacaaagttgctggattgggtggccacacagatggtaacttcttgacttttatatcgcaaaatcaagtcaatggattgcaaatcaacaaaaatggagaatggattgatgtgaatatttcaccaaattcttatgttgttttggctggtgattccttcaaagcttggacaaatggtcgattgcattctcctcttcacagagtaacaatgtccggagaaaatgatagactctccattcaattattttcattatcaaaaccaggtcacttcatcgaggcaccaaaagaactagtggatgaagaacaccctttactcttcaagccatttgaaattattggattatttgagtatggtaccacagaagctggctatacagctcctccaagtgatcttctcaagagttattgcggtgtttgatatgctaattgcgaatttccgcttcagcaaccaacttttctaataagtttcgtctgaaattcgtgttgttttaattattatgcattttatgtttgaattgttgtagttggcaattcatgtttaatttgtttgtgttttttttttttctttagtggaaatgat

SEQ ID NO: 27 - protein, 321 aa, Solanum lycopersycum
MASIKSVKVPTIDFSNYQELKPNTPLWESTKIQVFEAFQEYGCFEAIYDKVPNEIREETFDMSKEIFEFPLDTKVKNISEKPMHGYMGMIPQLPLYESLCIPDLLNPQSLQNFANIFWPQGNQHFCNLVKSYSNPLVELDEILKRMISENLRLKIHIDELLNANYFLFRFTHYKGSSITGGDENNKVAGLGGHTDGNFLTFISQNQVNGLQINKNGEWIDVNISPNSYVVLAGDSFKAWTNGRLHSPLHRVTMSGENDRLSIQLFSLSKPGHFIEAPKELVDEEHPLLFKPFEIIGLFEYGTTEAGYTAPPSDLLKSYCGV

SEQ ID NO: 28 - DNA, 963 bp, synthetic construct
  misc_feature 1..963: note = CDS of GAME31
  source 1..963: mol_type = other DNA
atgggatctaccaaatcaattaaagttcccactatcgatttttccaaccatcaagatctaaaaccaaacactccacaatgggaatccacaaaagatcaagtttttgaagcttttcaagaatttggttgttttgaagcaatatatgataaagtgccaaatgaaattagaaagggcatgtttgatgtttcaaaagaaatatttgaatttcccctagagaccaaattgaaaaacttatcagacaaaccattacatggctacatggggatgattccaaacttgcctttgtatgagagtttgtgtattcctgatttgcttaatcctcaaagtcttcaaaattttgaaaatatcttttggccacatggaaatcctgatttttgcaatttggtaaaatgttactcaaatccacttgtggaattggatgaaatgttgaagaggatgattttggagaaattgggagtagaaaatcagattgatgagttattggatcccaaatatgtcctatttagatttacacactacaaggggtcatcaccaactaatggagataaaaatactaaaagtgagggactaggtggccacactgatggtaacttcttgacttttatagcacaaaatcaagtaagtggattgcaaattaataaaaatggagagtggattgatgtcaacatctcaccaaattcttttgctgttttgtctgctgattccttcaaagcatggacaaatggtcgattgcattctccaattcacagagtaacaatggctggagaaaatgatagattctccattcaattattttcactatccaaaccaggtcacttcatagaggccccaaaagaacttgtggatgaacaacaccctttactcttcaaaccatatgaaatgcttggattatttaagtatgttacttcacaaagtggatatggagctcctggtgatgctttcaaggcttattgtggtgtttga

SEQ ID NO: 29 - protein, 320 aa, Solanum melongena
MGSTKSIKVPTIDFSNHQDLKPNTPQWESTKDQVFEAFQEFGCFEAIYDKVPNEIRKGMFDVSKEIFEFPLETKLKNLSDKPLHGYMGMIPNLPLYESLCIPDLLNPQSLQNFENIFWPHGNPDFCNLVKCYSNPLVELDEMLKRMILEKLGVENQIDELLDPKYVLFRFTHYKGSSPTNGDKNTKSEGLGGHTDGNFLTFIAQNQVSGLQINKNGEWIDVNISPNSFAVLSADSFKAWTNGRLHSPIHRVTMAGENDRFSIQLFSLSKPGHFIEAPKELVDEQHPLLFKPYEMLGLFKYVTSQSGYGAPGDAFKAYCGV

SEQ ID NO: 30 - DNA, 2345 bp, Solanum tuberosum
  source 1..2345: mol_type = other DNA
gaaactttgaagtctttcttgtttcctaaatattcctcaaatggcatctaccaaagttacgattcccaccatagatttttgcgattctgagcttaaaccaaacactccacaatgggaatcaacaaaagttcaagtttttgaagccttacaagaatttggttgttttgaagcaatatataacaaagttccaaatgaaattagagagggcatgtttgatactttaaaagaagtatttgattttccactgcccaaattgatagaatatagagagaaaccctttcatatatatgatgggcaaattccaagtgtaccactctttggtagtgtgtactctgctgatttggtcctcccaaatagtgttgaaacatttgccaataccttttggtctcatggaaaccctaattttaggtatgcattacttctttttcattaattatagggagtcacgatagtgtaagatgcattaaaaggagaaacgtttcctagtagaattgtttctattcctagggctagaatcaggaacctttagttaaattaatagagataatattcattccatcactaaaggtgaaaattaagtatcttatattgtccataaattttatatagaagagatgtgagaattaataaaataaaaattaaaaactcacgagtaaacaaaataattatatctaatttatattaataaagaagagtatttgattattatattaagtcaaatgataagctaataaatcaatattaacaatctaatcacatgatttatataaaattggttatgggtatgggaagggagggagggaagtacatttcattgaggaacaatgcaatagttagacaggatttaacatacttgaacaagatatcataatctaaaatgattaaaaataattttttaatattatctacacatcgcgcgaatatatatatatatatatattaagtgtatttcttaaataatattgtattactatttatataaattttgtatgttttaattttgcagcaatgtggcaaagtcctacttcaagcaacttatggaattaaatgacatggttaaaaagatggttttggagagtcttgggctaaaaaattacattgatgaattcttgaattccaatgtttatatgtcaagatttactaattacaaggtaattaaaggtgaaaatgagaataaatcaggattaccttcccacacagatagttcctacttgaccataattaaacaaaatcaaaatggattgcaagttctctacaaaaatggagagtggattgagctcaatcgtcaaaatggactgcaagttctctacaaaaatggagagtggattgagctcaatcatacttcaccaaattcctatattgttttatcagaagatgtttttatggtaagttattatttattttttattacagaagtcaaaaatacacctaaactttttatttatatgtatttttgacgcttaactctttatttttttgtgtgtaggggtggtttgttgctatagtagaggagaataaaagaaatagattttttttgtatgattgattattcaagcccaactagaagctaagattagaggagttttgaagcaacgaaaaaaaatgttgtgtgtgatttatagatattgatgcaggctcgatccgtgaaagaaatcactaatatttatattagattagatcgtttacctaactaaacatcccttgaagtactgccctttctccaaaccatatgtgaacgtcaaatattttatgcatcaacctgtctttttttatttggccccaactaacttcaatccacataaattattaaatcttgatattagttggaataacatatctcttttctgagaaattgaaaataatgccagaactatcataatctttttttaaaaaaattgtcttgttattatcttattaatttaaaattttctttcttcagaggaaatttaagtcaatctttttgttccttaattattaattaaacaaataaattcttatacatactttttatgtgttgatgctatgaattaattatacaggcatggacaaatgatagattgacatctgctcaacacagggttgtaacaacaggagacaaagaaagattctctattcaagttttttcctttccaaatccagattacactgtgaaggtcccacaagaattagtggatgaagaacaccctttaatgtacaagccttttaagatgtctgaatataataaatatattatgttaggtgctaaaaatggattgggtgtcaagaattattgtggtctttaaaaatttagtagctatgaaaatttatttatgtattgttttgatgaataaaatgtatcagatggc

SEQ ID NO: 31 - DNA, 963 bp, synthetic construct
  misc_feature 1..963: note = cDNA of GAME31of Solanum tuberosum
  source 1..963: mol_type = other DNA
atggcatctaccaaagttaagattcccaccatagatttttctaatctagaactaaaaccaaacactccactatgggaatccacaaaagttcaagtttttgaagctttaaaagaatatggttgttttgaagcaacatatgataaaattccaaatgaaattagagagggtatttttggtattacaaaagaaatatttcaatttcctttagagaccaaagtgaaaaattattcagatataacattacatggctatgtaggaatgattccacacttgccattttatgagagtttgtgtattcctgatttgcttaatcctcaaaatgttgaaacttttgctaatatcttttggcctcatggtaatcctgatttctgcaatttggtaaaagcttactcaaatccacttatggaattggatgaaatgttgaaaaagatgattttggagaatttgggattagaaaatcatattgatgaattgctggatattaattatatgagatttagatttacacattacaagggatcatcaattattagtggagatcatgaaaataatattaaacaagatggattgaatggccacacagatggtaacttcttgacttttatatcacaaaatcaagtcaatggtttgcaaatcaacaaaaatggagagtggattgatgtcaatatttcaccaaattcttatgttgttttgtctggtgattcattcaaagcatggacaaatggtcgattgcattctcccatccacaaggtaaaaatatttggtgaaagtgatagattctcaattcaattattttcattctcaaaaccaggtcactttataaaggccccaaaagaacttgtggatgaagaacaccctttactcttcaagccatttgaaatggttggattatctgagtatgttacttcccaagctggctatgcagctcccagtgatgctttcaaggcttattgtggtctttga

SEQ ID NO: 32 - protein, 320 aa, Solanum tuberosum
MASTKVKIPTIDFSNLELKPNTPLWESTKVQVFEALKEYGCFEATYDKIPNEIREGIFGITKEIFQFPLETKVKNYSDITLHGYVGMIPHLPFYESLCIPDLLNPQNVETFANIFWPHGNPDFCNLVKAYSNPLMELDEMLKKMILENLGLENHIDELLDINYMRFRFTHYKGSSIISGDHENNIKQDGLNGHTDGNFLTFISQNQVNGLQINKNGEWIDVNISPNSYVVLSGDSFKAWTNGRLHSPIHKVKIFGESDRFSIQLFSFSKPGHFIKAPKELVDEEHPLLFKPFEMVGLSEYVTSQAGYAAPSDAFKAYCGL

SEQ ID NO: 33 - DNA, 2345 bp, Solanum tuberosum; identical to SEQ ID NO: 30
  source 1..2345: mol_type = other DNA

SEQ ID NO: 34 - DNA, 990 bp, synthetic construct
  misc_feature 1..990: note = cDNA of GAME31-like1of Solanum tuberosum
  source 1..990: mol_type = other DNA
atggcatctaccaaagttacgattcccaccatagatttttgcgattctgagcttaaaccaaacactccacaatgggaatcaacaaaagttcaagtttttgaagccttacaagaatttggttgttttgaagcaatatataacaaagttccaaatgaaattagagagggcatgtttgatactttaaaagaagtatttgattttccactgcccaaattgatagaatatagagagaaaccctttcatatatatgatgggcaaattccaagtgtaccactctttggtagtgtgtactctgctgatttggtcctcccaaatagtgttgaaacatttgccaataccttttggtctcatggaaaccctaattttagcaatgtggcaaagtcctacttcaagcaacttatggaattaaatgacatggttaaaaagatggttttggagagtcttgggctaaaaaattacattgatgaattcttgaattccaatgtttatatgtcaagatttactaattacaaggtaattaaaggtgaaaatgagaataaatcaggattaccttcccacacagatagttcctacttgaccataattaaacaaaatcaaaatggattgcaagttctctacaaaaatggagagtggattgagctcaatcgtcaaaatggactgcaagttctctacaaaaatggagagtggattgagctcaatcatacttcaccaaattcctatattgttttatcagaagatgtttttatggcatggacaaatgatagattgacatctgctcaacacagggttgtaacaacaggagacaaagaaagattctctattcaagttttttcctttccaaatccagattacactgtgaaggtcccacaagaattagtggatgaagaacaccctttaatgtacaagccttttaagatgtctgaatataataaatatattatgttaggtgctaaaaatggattgggtgtcaagaattattgtggtctttaa

SEQ ID NO: 35 - protein, 329 aa, Solanum tuberosum
MASTKVTIPTIDFCDSELKPNTPQWESTKVQVFEALQEFGCFEAIYNKVPNEIREGMFDTLKEVFDFPLPKLIEYREKPFHIYDGQIPSVPLFGSVYSADLVLPNSVETFANTFWSHGNPNFSNVAKSYFKQLMELNDMVKKMVLESLGLKNYIDEFLNSNVYMSRFTNYKVIKGENENKSGLPSHTDSSYLTIIKQNQNGLQVLYKNGEWIELNRQNGLQVLYKNGEWIELNHTSPNSYIVLSEDVFMAWTNDRLTSAQHRVVTTGDKERFSIQVFSFPNPDYTVKVPQELVDEEHPLMYKPFKMSEYNKYIMLGAKNGLGVKNYCGL

SEQ ID NO: 36 - DNA, 1897 bp, Solanum tuberosum
  source 1..1897: mol_type = other DNA
ttattatttgcacaaaaaatacaaacaaagcatgaattcccatcgaaattactcactgttacaacaattcaaacataagatacacactactaaagaaacacgaatttcgacaagcattctgttagaaatcccatatatacttacagtattctaacaagaacgttcataaaaaaatcacgtttttttattctagcatatataaaacaaagaactctaaagctaaagatacacactattataaaaacacgaattccaaatgaaatccattggaaatgatgaagacattttcgatgaatattctgttagaaatcccaaatatactaacagtactctgacaaaaatgttcattagaaattcacgtttatcatatcaaagaccacaataagccttgaaagcatcactgggagctgcatagccagcttgggaagtaacatactcagataatccaaccatttcaaatggcttgaagagtaaagggtgttcttcatccacaagttcttttggggcctttataaagtgacctggttttgagaatgaaaataattgaattgagaatctatcactttcaccaaatatttttaccttgtggatgggagaatgcaatcgaccatttgtccatgcctgtataaattcacgtcgtcagtgcataaaactcaaacacatttatttgaaggatccaacatttttagagattcaaaaagcatagactccaacaaatatcaaaattcatttttcagttttgcatgaaaatattaaatatgtaggtagttccatttaatattcgagaaacataggttaattccaacaaatatgaagattcattttcaattttgcatcaagatattaaacctaaattttgtttggtatattccaaccttggaaatattcttcacaaatatcgttaggtatgcgtcagatcctctaaaatctatattttgtttttgaaggtgcaataataatatttttgaagagttcgagtaacatggatttcaacaaagtaatatgactagctaaaaaaataaaatgagtaacacttactttgaatgaatcaccagacaaaacaacataagaatttggtgaaatattgacatcaatccactctccatttttgttgatttgcaaaccattgacttgattttgtgatataaaagtcaagaagttaccatctgtgtggccattcaatccatcttgtttaatattattttcatgatctccactaataattgatgatcccttgtaatgtgtaaatctaaatctcatataattaatatccagcaattcatcaatatgattttctaatcccaaattctccaaaatcatctttttcaacatttcatccaattccataagtggatttgagtaagcttttaccaaattgctgcaaaaatttatcactatctcaaaaataactttctcgctactccacgactctaatcaatgcacaaaataattttattttaaaaaataaaataaagtagacataccagaaatcaggattaccatgaggccaaaagatattagcaaaagtttcaacattttgaggattaagcaaatcaggaatacacaaactctcataaaatggcaagtgtggaatcattcctacatagccatgtaatgttatatctgaataatttttcactttggtctctaaaggaaattgaaatatttcttttgtaataccaaaaataccctctctaatttcatttggaattttatcatatgttgcttcaaaacaaccatattcttttaaagcttcaaaaacttgaacttttgtggattcccatagtggagtgtttggttttagttctagattagaaaaatctatggtgggaatcttaactttggtagatgccatttgaaagaaacaaagaaggaattaaagacttcacaatgtgaa

SEQ ID NO: 37 - DNA, 339 bp, synthetic construct
  misc_feature 1..339: note = cDNA of GAME31-like2of Solanum tuberosum
  source 1..339: mol_type = other DNA
atgattccacacttgccattttatgggagtttgtgtattcctgatttgcttaatcctcaaaatgttgaaacttttgctaatatcttttggcctcatggtaatcctgatttctgcaatttggtaaaagcttactcaaatccacttatggaattggatgaattgttgaaaaggatgattttggagaatttgggattagaaaatcatattgatgaattgttggatcctaattatatgagatttagatttacacattacaagggatcatcaattattagtggagatcatgaaaataatattaaacatgatggattgaatgccacacagatggtagcttcttga

SEQ ID NO: 38 - protein, 112 aa, Solanum tuberosum
MIPHLPFYGSLCIPDLLNPQNVETFANIFWPHGNPDFCNLVKAYSNPLMELDELLKRMILENLGLENHIDELLDPNYMRFRFTHYKGSSIISGDHENNIKHDGLNATQMVAS

SEQ ID NO: 39 - DNA, 3623 bp, Solanum tuberosum
  misc_feature 677..1284: note = n is a, c, g, or t
  misc_feature 1884..1901: note = n is a, c, g, or t
  source 1..3623: mol_type = other DNA
attttttaataaaaataatacagtacaatacattacaatacaacgcaacacaatacaatacgttatgtaatcatatgcaataaccattcaaatataaattttcaaccacccatacatacgatacattttattcataaagaaaatacacatatataaattttcataccctacaaaaattttaaagaccacaataattcttgagattaattccatttttatcacctgacatagtttatttatgaaattcaagcaagttaaaaggcttgaagagtaaagggtggtcttcatccactaattcttttggggtccttcacagtataatctggatgtggtatggaaaataattgaatagataatctatctttgtctcctgttggtactactctgtgttcagcagatgtcaaactattatttgtccatgcctgtataaatccacaacatcgacacataaaaagcattagtgatttctttcacagagaaagggcagcacctcaaggggatgttaggaaaacaatctaatctaatagaaaatattagtgattttttctcgatcaagcccgcatcgtaatctatatatcacatacaaacaatcttatcgttacttcaaaactgctctgatcttagcttctagttgggcttaaataatcaaccatacaaaaaaaatctctatttctttnnnnnnnnnnnnnnnnnnnnnnnnnnnnnnnnnnnnnnnnnnnnnnnnnnnnnnnnnnnnnnnnnnnnnnnnnnnnnnnnnnnnnnnnnnnnnnnnnnnnnnnnnnnnnnnnnnnnnnnnnnnnnnnnnnnnnnnnnnnnnnnnnnnnnnnnnnnnnnnnnnnnnnnnnnnnnnnnnnnnnnnnnnnnnnnnnnnnnnnnnnnnnnnnnnnnnnnnnnnnnnnnnnnnnnnnnnnnnnnnnnnnnnnnnnnnnnnnnnnnnnnnnnnnnnnnnnnnnnnnnnnnnnnnnnnnnnnnnnnnnnnnnnnnnnnnnnnnnnnnnnnnnnnnnnnnnnnnnnnnnnnnnnnnnnnnnnnnnnnnnnnnnnnnnnnnnnnnnnnnnnnnnnnnnnnnnnnnnnnnnnnnnnnnnnnnnnnnnnnnnnnnnnnnnnnnnnnnnnnnnnnnnnnnnnnnnnnnnnnnnnnnnnnnnnnnnnnnnnnnnnnnnnnnnnnnnnnnnnnnnnnnnnnnnnnnnnnnnnnnnnnnnnnnnnnnnnnnnnnnnnnnnnnnnnnnnnnnnnnnnnnnnnnnnnnnnnnnnnnnnnnnnnnnnnnnnnnnnnnnnnnnnnnnggtgtgtttggtacgaaggaaaatattttctggaaaatgttttttaatttcccatgtttggttgactttaattatttggaaaatgttttccaaatcaacttattttcctcaaatttaaggaaaatgatttcccttaaaaattaaggaaaacattttcgaaacttctacttcatccttaaattataatatttttttacccctactaccaaaccagcccgccacccctgtcaaattttattttatttaaaaaattacttttgaaaaatatttcagggtcggaagtttggctggggtcctaggtcagatctctaggtcggattttgaacggtcatcaaggtcatgtcctagttcgggtgttagggtcgggtcctagattgattattgggattgattttcgagttaaaagttattttcctaaagagtattttctagtcttaagcgaaaaataaaagatattttctggaaaaaaaattcattcaccaaccaaacattaaaaaatagtttctactcatcaactaaatatgagaaaataagttagaaatccacttgttttccaagaaaacattttccttcataccaaacacacccttaatatatatnnnnnnnnnnnnnnnnnnttatatatgtatagatagctagtatacatactcgagcgatgtgcggaaaatattaatatgttatttttaatcttacccctacccatgcccctacccgaccttccccattcaaaaaaataaattaaaatttttaaaatttcaaatatatttttatcactaccaccaaactagctcccccgcccccctcccctcaaacataaaaaaaaaaaattaaaattatttttgaaaaatttttaaatcttaaattttttttacctcaccaacccctaccacccctactcccttccccctcatttttaatttcccatgtttggttgactttaatgatttggaaaatgttttccaaatcaacttattttcctcaaatttaaggaaaatgattatcctaaaagttattttcctaaagagtattttctagtctcaagagaaaataaaagatattttttcagaaaataattttcattcaccaaccaaacatgagaaaataagttagaaatccacttgttttccaagaaaacattttccttcataccaaacacacccttaatatataatgtatatatacctagtatacatactcgcgtgatgtgtgaaaaatatttaaatgttattttaaatcattttagattgtgatatcttgttcgagcatgttaaatcacgtccaactattgcattgttactcaatgaaatgtactcccctccatcccttcacatacccgtaaccaattctatatgaatagcgacaatgaatcatgtgattagattgttagtattgattttattagcttatcacttggatataattattaaatactcttctaattaatataaattagatatatttattttgtttactcgtgagttcttaatttttattttattaatgatcacatctcttttatataaaatgtatggacaataagatacttaattttcacctttagtgatggaatgaatattatctctataatttaactaaagattcatgattctagccttaggaataaaaacaattctagtaggaaacgtttctccttttaatgtgtcttacactatcgtgactccatattattaatctgaatcccaaaataaataccgaatacataatgaaaaaaaaaaaatctcctacaaatatatgagcaagaataattggtgtactaacatgactaaaactaaatgatatcacctacataaatcttattctttcaaatatcattaatgaaaaatgactttcataataccgagcacattatatgtaattaaaagaagtaatacatacctaaagttagggtttccatcagaccaaaaggtattggcaaatgtttcaatactatttgggaggaccaaatcagcagagctcacactaccatagagtggtatacttggaattttcccatcatatatatgaaagggtttttctctatattctatcaatttggacaatggaaaatcaaatacttcttttaaattatcaaacatgccctctctaatttcatttggaactttgtcatatattgcttcaaaacaaccaaattcttttaaggcttcaaaaacttgaacttttgttgattcccattgtggagtgtttggttttagctcaagattgcaaaaatctatggtgggaatcttacctttagtagatgccattgatgaataaattaaaaagagaggaaatagaaagaaataaagaaggagaaatactttacaatatgaaaattaaag

SEQ ID NO: 40 - DNA, 432 bp, synthetic construct
  misc_feature 1..432: note = cDNA of GAME31-like3of Solanum tuberosum
  source 1..432: mol_type = other DNA
atggcatctactaaaggtaagattcccaccatagatttttgcaatcttgagctaaaaccaaacactccacaatgggaatcaacaaaagttcaagtttttgaagccttaaaagaatttggttgttttgaagcaatatatgacaaagttccaaatgaaattagagagggcatgtttgataatttaaaagaagtatttgattttccattgtccaaattgatagaatatagagaaaaaccctttcatatatatgatgggaaaattccaagtataccactctatggtagtgtgagctctgctgatttggtcctcccaaatagtgttgaaacatttgccaataccttttggtctgatggaaaccctaactttaggtatgtattacttcttttaattatatataatgtgcttggtattatgaaagtcatttttcattaa

SEQ ID NO: 41 - protein, 143 aa, Solanum tuberosum
MASTKGKIPTIDFCNLELKPNTPQWESTKVQVFEALKEFGCFEAIYDKVPNEIREGMFDNLKEVFDFPLSKLIEYREKPFHIYDGKIPSIPLYGSVSSADLVLPNSVETFANTFWSDGNPNFRYVLLLLIIYNVLGIMKVIFH

SEQ ID NO: 42 - DNA, 2345 bp, Solanum tuberosum; identical to SEQ ID NO: 30
  source 1..2345: mol_type = other DNA

SEQ ID NO: 43 - DNA, 852 bp, synthetic construct
  misc_feature 1..852: note = cDNA of GAME31-like4of Solanum tuberosum
  source 1..852: mol_type = other DNA
atggcatctaccaaagttacgattcccaccatagatttttgcgattctgagcttaaaccaaacactccacaatgggaatcaacaaaagttcaagtttttgaagccttacaagaatttggttgttttgaagcaatatataacaaagttccaaatgaaattagagagggcatgtttgatactttaaaagaagtatttgattttccactgcccaaattgatagaatatagagagaaaccctttcatatatatgatgggcaaattccaagtgtaccactctttggtagtgtgtactctgctgatttggtcctcccaaatagtgttgaaacatttgccaataccttttggtctcatggaaaccctaattttagcaatgtggcaaagtcctacttcaagcaacttatggaattgaatgacatggtggaaaagatggttttggagagtcttgggctaaaaaattacactgatgaattcttgaattccaatgtttatatgtcaagatttactaattacaaggtaattaaaggtgaaaatgagaataaatcagcattaccttcacacacagatagttcctacttgaccataattaaacaaaatcaaaatggattgcaagcatggacaaatgatagattgacatctgctcaacacagggttgtaacaacaggagacaaagatagattctctgttcaattattttccctcctaaatccagattatactgtgaaggtcccaaaagaattagtggatgaagaacaccctttaatgtacaagccttttaagatgcctgaatataataaatatcttatgttaggtgctaaaaatggattgggtgtcaagaattattgtggtctttaa

SEQ ID NO: 44 - protein, 168 aa, Solanum tuberosum
MISCSGLKNYIDEFLNSNVFMSRFTNYRVIKGENENKSALPSHTDSSYLTIIKQNQNGLQVLYKNGEWIELNHTSPNSYIVLSEDVFMAWTNDRLTSAQHRVVTTGDKDRFSIQVFSFPNPDYTVKVPQELVDEEHPLMFKPFKLPEFNKYIKLGAKNGPGLKNYCGF

SEQ ID NO: 45 - DNA, 2345 bp, Solanum tuberosum; identical to SEQ ID NO: 30
  source 1..2345: mol_type = other DNA

SEQ ID NO: 46 - DNA, 507 bp, synthetic construct
  misc_feature 1..507: note = cDNA of GAME31-like5of Solanum tuberosum
  source 1..507: mol_type = other DNA
atgatatcttgttctgggctaaaaaattacattgatgaattcttgaattccaatgtttttatgtcaagatttactaattacagggtaattaaaggtgaaaatgagaataaatcagcactaccttcccacacagatagttcctacttgaccataattaaacaaaatcaaaatggattgcaagttctctacaaaaatggagagtggattgagctcaatcatacttcaccaaattcctatattgttttatcagaagatgtttttatggcatggacaaatgatagattgacatctgctcaacacagggttgtaacaacaggagacaaagatagattctctattcaagttttttcctttccaaatccagattacactgtgaaggtcccacaagaattagtggatgaagaacaccctttaatgttcaagccttttaagttgcctgaatttaataaatatattaagttaggtgctaaaaatggaccgggtctcaagaattattgtggtttttaa

SEQ ID NO: 47 - protein, 168 aa, Solanum tuberosum; identical to SEQ ID NO: 44

SEQ ID NO: 48 - DNA, 2762 bp, Solanum tuberosum
  source 1..2762: mol_type = other DNA
cactaatatatttttaataaaaacaatacagtacaatacattacaatacaacgcaacacaacacaatacaatacgttatgaaatcatatgcaataaccacacaaatataaattttcaaccacccatgcatacgatacattgtattcataaagaaaatacacataaataaataccctactaaatttttaaagaccacaataattcttgagattaattcaatttttattacctgacatagtttatttatgaaattcaagcaagttaaaaggcttgaagagtaagggtggtcttcatccactaattattttggggccttcacagcaaaatcttgatttgggaaaggaaaataattgaatagatagtctatctttgtctcctgttgttactactctgtgttcagcagatgtcaaactatcatttgtccatgcctgtataaatccacaacatcgacacataaaaagtattagtgatttcttttcacagagaaagggcaacacctcaagggatgttaggaaaacaatctaatctaatacaaaatattagtgattttttctcgatcaagcccgcatcgtaatctataaatcacatacaaacaatcttatcgttacttcaaaactgctctgatcttagcttctagttgggcttgaataatcaaccatacaaaaaaatctctatttcttttattctcctcttctatagcatcaacccaccccctcacacacaaaataataaagagttaagcgtcaaaaatacacataaataaataatttaggtgtattttttaccttgatactcaaaaataaataataacttaccctgaaagcatctgctgataaaacaatataggaatttggtgttgtattattgagctctatccactctccatttttgtagagaacttgcaatccattttgattttgtttaattatagtcaagtagccactatctgtgtggggaggtaattctgatctattctcatcttcacctttaattaccttgtaattagtaaatcttgacacaaaaacattggaattcaagatttcatcaatgtaatttgttttcccaagactctccaaaaccattttttccaccatgtcattcaattccataagttgcttgaagtaggactttgccacattgctgccaaattaaaacatacaaaacttatataatggtaatgcaatattgtgatattactcaaaattatgtaagaaatacacttagggtgtgtttggtacgaaggaaaatattttctagaaaatgttttttaatttcccatgtttggttgactttaatgatttggaaaatgttttccaaatcaacttattttcctcaaatttaaggaaaatgattatcctaaaagttattttcctaaagagtattttctagtcttaagtgaaaaataagttagaaatccacttgttttccaagaaaacattttccttcataccaaacacacccttaatatataatgtatatatacctagtatacatactcgcgcgatgtgtgaaaaatatttaaatgttattttaatcattttagattgtgatatcttgttcgagcatgttaaatcatgtccaactattgcattgttactcaatgaaatgtactcccctccatcccttcacatacccgtaaccaattctatatgaatagcgatgtgtgaaaaatatttaaatgttatttttaatcattttagattgtgatatcttgttcgagcatgttaaatcatgtccaactattgcattgttactcaatgaaatgtactcccctccatcccttcacatacccgtaaccaattctatatgaatagcgacaatgaatcatgtgattagattgttaatattgattttattagcttatcacttggatataattattaaatactcttctaattaatataaattagatatatttattttgtttactcgtgagttcttaatttttattttattaatgatcacatctcttttatataaaatgtatggacaataagatacttaattttcacctttagtgatggaatgaatattatctctataatttaactaaagattcctgattctagccttaggaataaaaacaattctagtaggaaacgtttctccttttaatgtgtcttacactatcgtgactccatattattaaatctgaaatcccaaaaataaataccgaatacataatgaaaaaaaaaaaatctcctacaaaatatatgagcaagaataattggtgtactaacatgactaaactaaatgatatcacctacataaatcttattctttcaaatatcattaatgaaaaataactttcataataccgaacacattatatataattaaaagaagtaatacatacctaaagttagggtttccatcagaccaaaaggtattggcaaatgtttcaacactatttgggaggaccaaatcagcagagctcacactaccatagagtggtatacttggaatttgcccatcatataaatggggtttttctctatattctatcaatttggacactggaaaatcaaatacttcttttaaagtatcaaacatgccctctctaatttcatttggaactttgtcatatattgcttcaaaacaaccaaattcttttaaggcttcaaaaacttgaacttttgttgattcccattgtggagtgtttggttttagctcaagattgcaaaaatctatggtgggaatcttaactttggtagatgccattgatgaataaattaaatagagaggaaatagaaagaaataaa

SEQ ID NO: 49 - DNA, 828 bp, synthetic construct
  misc_feature 1..828: note = cDNA of GAME31-like6 of Solanum tuberosum
  source 1..828: mol_type = other DNA
atggcatctaccaaagttaagattcccaccatagatttttgcaatcttgagctaaaaccaaacactccacaatgggaatcaacaaaagttcaagtttttgaagccttaaaagaatttggttgttttgaagcaatatatgacaaagttccaaatgaaattagagagggcatgtttgatactttaaaagaagtatttgattttccagtgtccaaattgatagaatatagagaaaaaccccatttatatgatgggcaaattccaagtataccactctatggtagtgtgagctctgctgatttggtcctcccaaatagtgttgaaacatttgccaataccttttggtctgatggaaaccctaactttagcaatgtggcaaagtcctacttcaagcaacttatggaattgaatgacatggtggaaaaaatggttttggagagtcttgggaaaacaaattacattgatgaaatcttgaattccaatgtttttgtgtcaagatttactaattacaaggtaattaaaggtgaagatgagaatagatcagaattacctccccacacagatagtggctacttgactataattaaacaaaatcaaaatggattgcaagttctctacaaaaatggagagtggatagagctcaataatacaacaccaaattcctatattgttttatcagcagatgctttcagggcatggacaaatgatagtttgacatctgctgaacacagagtagtaacaacaggagacaaagatagactatctattcaattattttcctttcccaaatcaagattttgctgtgaaggccccaaaataattagtggatga

SEQ ID NO: 50 - protein, 275 aa, Solanum tuberosum
MASTKVKIPTIDFCNLELKPNTPQWESTKVQVFEALKEFGCFEAIYDKVPNEIREGMFDTLKEVFDFPVSKLIEYREKPHLYDGQIPSIPLYGSVSSADLVLPNSVETFANTFWSDGNPNFSNVAKSYFKQLMELNDMVEKMVLESLGKTNYIDEILNSNVFVSRFTNYKVIKGEDENRSELPPHTDSGYLTIIKQNQNGLQVLYKNGEWIELNNTTPNSYIVLSADAFRAWTNDSLTSAEHRVVTTGDKDRLSIQLFSFPKSRFCCEGPKIISG

SEQ ID NO: 51 - DNA, 1429 bp, Solanum tuberosum
  source 1..1429: mol_type = other DNA
gcagcaatgtggcaaagtcctacttcaagcaacttatggaattgaatggcatggtggaaaagatggttttggagagtcttgggctaaaaaattacattgatgaattcttgaattccaatgtttatatgtcaagatttactaattacaaggtaattaaaggtgaaaatgagaataaatcaggattaccttcccacacagatagttcctacttgaccataattaaacaaaatcaaaatggattgcaagttcttctacaaaaatggagagtggattgagctcaatcatacctcaccaaattcctatattgttttatcagcagatgctcttatggtaagttattatttatttttgattacagcagtcaaaaatacgcctaaacttctaatttatatgtatttttgacgctttaactcattattattttttgtgtgtggggtggtttgttgctatagtagaggagaataaaagaaatagagattttttttgtatgattgattattcaagcccaactagaagctaagattagaggagttttcaaccaacgaaaaaaatgtttgtgtgtgatttatatatcatgatgcaggctcaatccgtaaaagaaatcactaatatttgtattagattagattgtttacctaactaacatcccttgaagtgttgccctttctccaaaccctatgtgaacgtcaaatattttatgcatcaacctgtcttattttatttgacctcaactaacttcaatccacaaaaaatattaaatcttgatattatttggaataacgtatctctttttctggaaaattgaaaatgataccagaactatcataataattttttaaattgtcttgttattatcttattaatttaaaattttcattctccataggaaatttaagtcaatctttttgttccttaattattaattaaacaaataaattcttatacatactttttatgtgttgatgatatgaattaattatacaggcatggacaaatgatagattgacatctgctcaacatagggttgtaacaacaggagacaaagatagattctctgttcaattattttccctcgtaaatccagattatactttgaaggtcccaaaagaattagtggatgaagaacaccctttaatgtacaagccttttaagatgcctgaatataataaatatcttatgttaggtgctaaaaatggattgggtgtcaagaattattgtggtctttaaaaatttagtagctatgaaaatttatttatgtattgttttgatgaataaaatgtatcagatggctggttgaatactttgaatttatatttggatggttattacgtatgattgcgtaaagtattgtattgtattttattttgttgtgttgttttgtattgtgttgcgttgtatatattgttttgatgaataaaatatatgagtg

SEQ ID NO: 52 - DNA, 339 bp, synthetic construct
  misc_feature 1..339: note = cDNA of GAME31-like7 of Solanum tuberosum
  source 1..339: mol_type = other DNA
atggattgcaagttcttctacaaaaatggagagtggattgagctcaatcatacctcaccaaattcctatattgttttatcagcagatgctcttatggcatggacaaatgatagattgacatctgctcaacatagggttgtaacaacaggagacaaagatagattctctgttcaattattttccctcgtaaatccagattatactttgaaggtcccaaaagaattagtggatgaagaacaccctttaatgtacaagccttttaagatgcctgaatataataaatatcttatgttaggtgctaaaaatggattgggtgtcaagaattattgtggtctttaa

SEQ ID NO: 53 - protein, 112 aa, Solanum tuberosum
MDCKFFYKNGEWIELNHTSPNSYIVLSADALMAWTNDRLTSAQHRVVTTGDKDRFSVQLFSLVNPDYTLKVPKELVDEEHPLMYKPFKMPEYNKYLMLGAKNGLGVKNYCGL

SEQ ID NO: 54 - DNA, 55 bp, synthetic construct
  misc_feature 1..55: note = RF-Tomato-GAME31-Forward Primer
  source 1..55: mol_type = other DNA
tccgcgggtgaaaacctgtacttccagggtgcatctatcaaatcagttaaagttc

SEQ ID NO: 55 - DNA, 57 bp, synthetic construct
  misc_feature 1..57: note = RF-Tomato-GAME31-Reverse Primer
  source 1..57: mol_type = other DNA
gtggtggtgctcgagtgcggccgcaagctttcaaacaccacaataaatcttgaaaag

SEQ ID NO: 56 - DNA, 55 bp, synthetic construct
  misc_feature 1..55: note = RF-Eggplant-GAME31-Forward Primer
  source 1..55: mol_type = other DNA
tccgcgggtgaaaacctgtacttccagggtggatctaccaaatcaattaaagttc

SEQ ID NO: 57 - DNA, 51 bp, synthetic construct
  misc_feature 1..51: note = RF-Eggplant-GAME31-Reverse Primer
  source 1..51: mol_type = other DNA
gtggtggtgctcgagtgcggccgcaagctttcaaacaccacaataagcctt

SEQ ID NO: 58 - DNA, 149 bp, synthetic construct
  misc_feature 1..149: note = SlGAME31-RNAi
  source 1..149: mol_type = other DNA
gggtttcgttggaaattcgtcttgtttttttttttcaagtagtgtacatcttatttttggattgttgatgttgagcgctaatgtttaatttgtttgtgttttgaagaggatgattatactctttaagaggattcaccgtaatcttttag

SEQ ID NO: 59 - DNA, 966 bp, synthetic construct
  misc_feature 1..966: note = SlGAME31-Cosup
  source 1..966: mol_type = other DNA
atggcatctatcaaatcagttaaagttcctactatagatttttccaattatcaagagctaaaaccaaacactccactatgggaatccacaaaaattcaagtttttgaagctttacaagaatatggttgttttgaagcaatatatgataaagtttcaaaggaaattagagaggaaacatttgatatgtcaaaagaaatatttgaatttcctttagagactaaagtgaaaaatatctcagaaaaaccaatgcatggctatatggggatgattccacaattgccattgtatgagagtttgtgtattcctgatttgcttaatcctcaaagtcttgaaaaattttctaatatcttttggcctcagggtaatcaacatttctgcaatttgataaaatcttattctaatccacttgtggaattggatgggatgttgaaaaggatgatttcggagaatttgggattgaaaaatcacattgatgaattattgaatgccaattacttcctatttagatttacacattataagggatcatcaattgctagtggagatgaaaataataaagctgctggattgggtggccacacggatggtaacttcttgacttttatatcgcaaaatcaagttaatggattgcaaatcaacaaaaatggagaatggattgatgtgattatttcaccaaattcttacgttgttttggccggtgattccttcaaagcttggacaaatggtcgattgcattcacctctccacagagtaacaatgtccggacaaaatgatagactctccattcaattgttttcattatcaaagccaggtcacttcatccaggcaccaaaagaactagtagatgaagaacacccattactcttcaagccatttgaaattcttgaattattcaagtatggtaccacagaagctggctatacagctcctccaagtgatcttttcaagatttattgtggtgtttga

SEQ ID NO: 60 - DNA, 29 bp, synthetic construct
  misc_feature 1..29: note = qRT-PCR forward primer
  source 1..29: mol_type = other DNA
agtacaagtaatcacgttggttcctatga

SEQ ID NO: 61 - DNA, 34 bp, synthetic construct
  misc_feature 1..34: note = qRT-PCR reverse primer
  source 1..34: mol_type = other DNA
cactagaaagttttttactttataggtgaggaaa

SEQ ID NO: 62 - DNA, 35 bp, synthetic construct
  misc_feature 1..35: note = Cloning SlGAME31 for RNAi forward primer
  source 1..35: mol_type = other DNA
aaaaagcggccgcgggtttcgttggaaattcgtct

SEQ ID NO: 63 - DNA, 38 bp, synthetic construct
  misc_feature 1..38: note = Cloning SlGAME31 for RNAi reverse primer
  source 1..38: mol_type = other DNA
aaaaaggcgcgccctaaaagattacggtgaatcctctt

SEQ ID NO: 64 - DNA, 55 bp, synthetic construct
  misc_feature 1..55: note = Cloning SlGAME31 for Cosupression forward primer
  source 1..55: mol_type = other DNA
ggggacaagtttgtacaaaaaagcaggctatggcatctatcaaatcagttaaagt

SEQ ID NO: 65 - DNA, 54 bp, synthetic construct
  misc_feature 1..54: note = Cloning SlGAME31 for Cosupression reverse primer
  source 1..54: mol_type = other DNA
ggggaccactttgtacaagaaagctgggttcaaacaccacaataaatcttgaaa

SEQ ID NO: 66 - protein, 259 aa, S. lycopersicum
MASKLRLEGKVAIITGGASGIGEASARLFVQHGARVVVADIQDELGLQVVQSIGIHKATYRHCDVTDEKQVEDTVAYAVQKYATLDIMFSNVGTLNFCSVLDMDMTAFDETMTVNVRGSALAVKHAARVMVDKKIRGSIICNVSLEGILAGAASLAYIASKHAVVGIVKAAARELGPYGIRVNGVSPYGIATPLVCKAYGLDAAPLEAAINGNANLKGVTLSTMHVAQSALFLASDESAYTSGQNLAVDGGLSSILKLQ

SEQ ID NO: 67 - protein, 259 aa, S. pennellii
MASKLRLEGKVAIITGGASGIGEASARLFVQHGARVVVADIQDELGLQVVQSIGIHKATYRHCDVTDEKQVEDTVAYAVQKYATLDVMFSNVGTLNFCSVLDMDMTAFDETMTVNVRGSALAVKHAARVMVDKKIRGSIICNVSLEGILAGAASLAYIASKHAVVGIVKAAARELGPYGIRVNGVSPYGIATPLVCKAYGLDAAPLEAAINGNANLKGVTLSTMHVAQSALFLASDESAYTSGQNLAVDGGLSSILKLQ

SEQ ID NO: 68 - protein, 236 aa, C. annuum
LEGKVAVITGAASGIGEASARLFVEHGARVVIADIQDELGLQIAASIGTDKASYIHCDVTDEKQVEEAVAYAVENSVLDLDVKAFDETMVINARGSAVAVKHAARVMVEKKIRGSIICTASLEGILAGAASLAYVSSKHAVVGLVKAAARELGVHGIRVNGVSPYGIATPLVCKAYGLDAGPLETAIYGNAHLKGVTLSTMHVAQAALFLASDESAYISGQNLAVDGGLSSILKLE

SEQ ID NO: 69 - protein, 261 aa, N. benthamiana
MANKLRLEGKVAVITGGASGIGEATARLFVEHGARVVIADIQDELGLQVVASIGTDKASYRHCDVTDENKVEETVAYAVEKYGTLDIMFSNVGTLNFCSVLDIDVTAFDKTMALNVRGTALAVKHAARVMVAKQVKGSIICNASIEAILAGAASLAYVASKHAVVGIVKAAARELGLHGIRVNGVSPYGIATPLVCKAYGCEDAASLEAGISVNAHLKGVTLSTEHIAQAALFLASDESAYISGHNLAVDGGLTSMLKLSY

SEQ ID NO: 70 - protein, 258 aa, S. melongena
MANKLKLEGKVAVITGGASGIGEESARLFVEHGARVVIADIQDDLGLEVVTSIGADKACYRHCDVSEEKQVKETVAYAVEKYGTLDIMFSNAGTLGTLGSVLEMDMTAFDMTMAVNMRGSALAVKHAARVMVANKIRGSIICTASVEAILAGAAPLAYVASKHAILGVMKAAARELGQYGIRVNCVSPYGIATPLVCKAYHSDAGSLEASIYERAHLKGITLSTKHIANASLFLASDESAYVSGHNLAVDGALSSIMS

SEQ ID NO: 71 - protein, 263 aa, C. annuum
MIFFFCGTRLEGKIAIITGAASGIGEASARLFVEHGAHVIIADIQDELGLQVVSSIGTDKACYRHCDVTDEKQVEETVAYAVEKYGTLDIMFSNAGMLGTFGSLLDMDVKEFDLTIAVNTRGAALAVKHAARVMVAKNIRGSIICTASVESILAGAAPLAYIASKHGILGVVKAAARELGKNGIRVNCVSPFGIATPMVCKSYGAEASYIETSVGGHANLKGVSLTTKHIAEAALFLASEESAYISGQNLAVDGGLSAIMRLD

SEQ ID NO: 72 - protein, 260 aa, S. melongena
MANKLRLEGKVAVITGGASGIGEASARLFVEHGARVVIADIQDELSLQVVSSIGGDKACYRRCDVSDEKQVEETVAYAVEKYGTLDIMFSNAGILGSFGSLLEMDMTAFDRIMAVNTRGAALAVKHAARVMVANKIRGSIICTASVEAILAGEASLAYIASKHAILGVVKAAARDLGQYGIRVNCVSPYGIATPMVCKSIGADAATIEARICGNANLKGVSLNTKHIAEAALFLGSDESAYVSAHNLAVDGGLSSIMKLN

SEQ ID NO: 73 - protein, 262 aa, S. tuberosum
MANKLRLEGKVAVITGGASGIGEATARLFVEHGAHVVIADIQDELALQVVSSIGSDNVCYRRCDVTDEKQVDETVAFAVQKYGTLDIMFSNAGILGSSGSLLEMDMAVFDRTMAVNTRGAALAVKHAAKVMVAKKIRGSIICTASVESILAGAASLAYIASKHAVLGVVKAAARELGQHGIRVNCVSPFGVATPMVCKSFGADAAAMEATIRGNANLKGVSLTTMHIAEAALFLASDESAYISAHNLAIDGGLSSIMKINVN

SEQ ID NO: 74 - protein, 260 aa, S. lycopersicum
MANKLRLEGKVAVITGGASGIGEAAARLFVEHGARVVIADIQDELALQVASSIGSDNVCYQRCDVSDEKQVNETVAFAVEKYGTLDIMFSNAGILNPFESILEMDMTVFDRTIAVNARGAALAVKHAARVMVANKIRGSIICTASVESILAGAAPLAYIASKHAVLGVVKAAARELGQHGIRVNCVSPFGIATPMVCKSFGADAAAIEAKICGNANLKGVSLTTMHIAEAALFLASDESAYISAQNLAVDGGLSSMMKLM

SEQ ID NO: 75 - protein, 260 aa, S. pennellii
MANKLRLEGKVAVITGGASGIGEAAARLFVEHGARVVIADIQDELALQVASSIGSVNVCCRRCDVSDEKQVNETVAFAVEKYGTLDIMFSNAGILNPFESILEMDMTVFDRTIAVNARGAALAVKHAARVMVANKIRGSIICTASVESILAGAAPLAYIASKHAVLGVVKAAARELGQHGIRVNCVSPFGIATPMVCKSFGADAAAIEAKICGNANLKGVSLTTMHIAEAALFLASDESAYISAQNLAVDGGLSSMMKLM

SEQ ID NO: 76 - protein, 260 aa, N. benthamiana
MANKRRLEGKVAVITGAASGIGEATARLFVEHGARVVIADIQDELGHQVVASIGTDKASYRHCDVTDEKQVEDTVVYTVEKYGTLDIMFSNAGTIGTLGSILDMDMTVFDRTMAINARGSALAVKHAARVMVTKKIQGSIICTASLEATLAGAAPLAYVTSKHAILGVVKAAARELGQHGIRVNCVSPYGIATPMVCKTFGGDAAPIEASISGNANLKGITLSTKHIAEAALFLASDESAYVSAHNLAVDGGLSSIMKLD

SEQ ID NO: 77 - protein, 241 aa, N. benthamiana
MANKLRLEGKVAVITGAASGIGEATARLFVEHGARVVIADIQDELGHQVVASIGTDKASYRHCDVTDEKQVEDTVVYAVEKYGTLDIMFSNAGTIGTLSSILDMDMTVFDRTMAINARGSALAVKHAARIMVTKKIQGSIICTASLEAILAGAAPLAYVASKHAILGVVKAAARELGQHGIRVNCVSPYGIATPMVCKTFGGDAAPIEASISGNANLKGITLSTKHIAEAALFLASDESAY

SEQ ID NO: 78 - protein, 257 aa, A. thaliana
MSGKRLDGKIVIITGGASGIGAESVRLFTEHGARVVIVDVQDELGQNVAVSIGEDKASYYHCDVTNETEVENAVKFTVEKYGKLDVLFSNAGVIEPFVSILDLNLNELDRTIAINLRGTAAFIKHAARAMVEKGIRGSIVCTTSVAAEIAGTAPHGYTTSKHGLLGLIKSASGGLGKYGIRVNGVAPFGVATPLVCNGFKMEPNVVEQNTSASANLKGIVLKARHVAEAALFLASDESAYVSGQNLAVDGGYSVVKP

SEQ ID NO: 79 - protein, 266 aa, M. truncatula
MSRKRLEGKVAIVTGGASGIGAETAKTFVENGAFVVIADINDELGHQVATSIGLDKVSYHHCDVRDEKQVEETVAFALEKYGTLDIMFSNAGIEGGMSSSILEFDLNEFDNTMAINVRGSLAAIKHAARFMVERKIRGSIICTASVAASVAGNRGHDYVTSKHGLLGLVRSTCGELGAYGIRVNSISPYGVATPLACRALNMEMSKVEANMKDSANLKGITLKATHIAEAALFLASEESAYISGHNLVVDGGFSVINSCVPTTIKK

SEQ ID NO: 80 - protein, 266 aa, C. annuum
MAVVMQKLKGKVAIVTGGASGIGEATVRLFAEHGARAVVIADIQDEKGRAVAESIPLQVCSYVHCDVSDENQVKGLVDWTVKKYGQLDIMFSNAGTVGNSGQKVLDLDLSEFDRVIRVNARGMAACVKHAARAMVEQGGRGSIICTGSVGASKGAAWRTDYTMSKHAVLGLVTSASRQLGKYGIRVNSISPSAVMTPLMSSAEAETSMKVLKMYGPLTSLKGITLTVKHLADAVLFLASDDSAFVNGHDLLVDGGLLHLPDPMSSL

SEQ ID NO: 81 - protein, 266 aa, S. tuberosum
MAEVTQKLKGKVAIVTGGASGIGEATARLFAQHGARAVVIADIQDGKGRAVAVSIPSQICSYVQCDVSDENQVKAMVDWTVQKYGQLDIMFSNAGVVGNSGQKVLDLDLSEFDRVMNVNARGMAACVKHAARAMVDKRVRGSIICTGSIGASRGGAWRTDYIMSKHAVLGLVRSACRQLGEYGIRVNSISPSAVMTPLMISAEPEVSMKSLKRYGPQTSLKGITLTVKHLAEAALFLASDDSAFSSRSNEFIVKQREQPNLSLFFF

SEQ ID NO: 82 - protein, 266 aa, S. melongena
MSAITQKLNGKVAIVTGGASGIGEATVRLFAQHGARAVVIADIQDEKGRAVAQSIPSQICIYVKCDVSDENQVKSMVDWTVQQYGQLDIMFSNAGTVGNSGQKILDLDLSEFDRVMNVNARGMAACVKHAARAMVEKRVRGSIICTGSIAASRAGAWRTDYAMSKHAVLGLMRSASRQLGEYGIRVNSISPSAVMTPLMISAEAEASMRVLKMYGSVTSLKGITLTVKHLADAVLFLASDDSVFVSGHDLAVDGGLISLPDPMSSL

SEQ ID NO: 83 - protein, 302 aa, O. sativa
MFTAMHRILSRGRRTPAASSSSVTAFATASDSQRLAGKVAVITGGASGIGRATAEEFVRNGAKVILADVQDDLGHAVAAELGADAASYARCDVTDEAQVAAAVDLAVARHGRLDVVFNNAGIPGDLTPTPVGALDLADFDRVMAVNTRAVVAGVKHAARVMVPRRRGSIICTASTAGVIGGVAVPHYSVSKAAVLGLVRAVAGEMARSGVRVNAISPNYIWTPMAAVAFARWYPSRSADDHRRIVENDINEMDGVTLEAEDVARAAVFLASDEAKYVNGHNLVVDGGYTVGKVPNMPVPDGH

SEQ ID NO: 84 - protein, 300 aa, O. sativa
MFRAAQLLLRETNRALGAATSPAGFVSGFSTASNSAQRLAGKVAVITGGASGIGKATAKEFIENGAKVIMADVQDDLGHSTAAELGPDASYTRCDVTDEAQVAAAVDLAVKRHGHLDILYNNAGVMGAMPQDDMASVDLANFDRMMAINARAALVGIKHAARVMSPRRSGVILCTASDTGVMPMPNIALYAVSKATTIAIVRAAAEPLSRHGLRVNAISPHGTRTPMAMHVLSQMYPGVSKDDLEKMADAAMDAGEVMEPKYVARAALYLASDEAKYVNGHNLVVDGGFTSHKGSDTRLN

SEQ ID NO: 85 - protein, 285 aa, A. thaliana
MSTNTESSSYSSLPSQRLLGKVALITGGATGIGESIVRLFHKHGAKVCIVDLQDDLGGEVCKSLLRGESKETAFFIHGDVRVEDDISNAVDFAVKNFGTLDILINNAGLCGAPCPDIRNYSLSEFEMTFDVNVKGAFLSMKHAARVMIPEKKGSIVSLCSVGGVVGGVGPHSYVGSKHAVLGLTRSVAAELGQHGIRVNCVSPYAVATKLALAHLPEEERTEDAFVGFRNFAAANANLKGVELTVDDVANAVLFLASDDSRYISGDNLMIDGGFTCTNHSFKVFR

SEQ ID NO: 86 - protein, 275 aa, O. sativa
MAGSSYGDVHESARKLVGKVALITGGASGIGECTARLFVKHGAQVVVADIQDEAGARLCAELGSATASYVRCDVTSEDDVAAAVDHAVARYGKLDVMFNNAGIGGAACHSILESTKADFDRVLAVNLTGPFLGTKHAARVMVAAGRGGCIIGTASLASAVAGTASHAYTCAKRALVGLTENAAAELGRHGIRVNCVSPAAAATPLATGYVGLEGEAFEAAMEAVANLKGVRLRVEDIAAAVLFLASDDARYVSGHNLLIDGGCSIVNPSFGIFKD

SEQ ID NO: 87 - protein, 274 aa, O. sativa
MAAGSSHVSADARKLVGKVAVITGGASGIGACTARLFVKHGARVVVADIQDELGASLVAELGPDASSYVHCDVTNEGDVAAAVDHAVARFGKLDVMFNNAGVSGPPCFRMSECTKEDFERVLAVNLVGPFLGTKHAARVMAPARRGSIISTASLSSSVSGAASHAYTTSKHALVGFTENAAGELGRHGIRVNCVSPAGVATPLARAAMGMDDEAIEAIMANSANLKGAGALKADDIAAAALFLASDDGRYVSGQNLRVDGGLSVVNSSFGFFRD

SEQ ID NO: 88 - protein, 274 aa, O. sativa
MAGSSHVSADARKLVGKVAVITGGASGIGACTARLFVKHGARVVVADIQDELGASLVAELGPDASSYVHCDVTNEGDVAAAVDHAVATFGKLDVMFNNAGVTGPPCFRITESTKEDFERVLAVNLIGPFLGTKHAARVMAPARRGSIISTASLSSSVSGTASHAYTTSKRALVGFTENAAGELGRHGIRVNCVSPAAVATPLARAAMGMDMDDETIEAIMEKSANLKGVGLKVDDIAAAALFLASDDGRYVSGQNLRVDGGVSVVNSSFGFFRD

SEQ ID NO: 89 - protein, 349 aa, A. thaliana
MELINDFLNLTAPFFTFFGLCFFLPPFYFFKFLQSIFSTIFSENLYGKVVLITGASSGIGEQLAYEYACRGACLALTARRKNRLEEVAEIARELGSPNVVTVHADVSKPDDCRRIVDDTITHFGRLDHLVNNAGMTQISMFENIEDITRTKAVLDTNFWGSVYTTRAALPYLRQSNGKIVAMSSSAAWLTAPRMSFYNASKAALLSFFETMRIELGGDVHITIVTPGYIESELTQGKYFSGEGELIVNQDMRDVQVGPFPVASASGCAKSIVNGVCRKQRYVTEPSWFKVTYLWKVLCPELIEWGCRLLYMTGTGMSEDTALNKRIMDIPGVRSTLYPESIRTPEIKSD

SEQ ID NO: 90 - protein, 264 aa, A. thaliana
METDKRWSLAGKTALVTGGTRGIGRAVVEELAKFGAKVHTCSRNQEELNACLNDWKANGLVVSGSVCDASVRDQREKLIQEASSAFSGKLNILINNVGTNVRKPTVEYSSEEYAKIMSTNLESAFHLSQIAHPLLKASGVGSIVFISSVAGLVHLSSGSIYGATKGALNQLTRNLACEWASDNIRTNCVAPWYIKTSLVETLLEKKEFVEAVVSRTPLGRVGEPEEVSSLVAFLCLPASSYITGQVISVDGGFTVNGFSYAMKP

SEQ ID NO: 91 - protein, 310 aa, Z. mays
MDAAAAAASPTSKRIALVTGGNKGIGLETCRQLASRGVRVVLTARNEARGLEAVERVRCARGDAEVYFHQLDVTDPCSAARLADFVRDQFGRLDILINNAGISGVHRDPVLSAAVKDKVDGMDVNQRVEWMKENSKETYEEAVQCMKTNYYGAKLVTEALLPLLQLSSSGRIVNVSSGFGLLRNFNSEDLRKEFEDIDNLTESRLEELMDKFLEDFKANLVEEHGWPTGGSSAYKVVKAALNAYTRILAKKYPTLRINCLTPGYVKTDISMHMGVLTLEEGARNPVKVALLPDDGPTGAYFDLNGEASFV

SEQ ID NO: 92 - protein, 303 aa, A. thaliana
MAEETPRLFNGFCRYAVVTGANRGIGFEICRQLASEGIRVVLTSRDENRGLEAVETLKKELEISDQSLLFHQLDVADPASITSLAEFVKTQFGKLDILVNNAGIGGIITDAEALRAGAGKEGFKWDEIITETYELTEECIKINYYGPKRMCEAFIPLLKLSDSPRIVNVSSSMGQLKNVLNEWAKGILSDAENLTEERIDQVINQLLNDFKEGTVKEKNWAKFMSAYVVSKASLNGYTRVLAKKHPEFRVNAVCPGFVKTDMNFKTGVLSVEEGASSPVRLALLPHQETPSGCFFSRKQVSEF

SEQ ID NO: 93 - protein, 311 aa, P. bracteatum
MPETCPNTVTKMRCAVVTGGNKGIGFEICKQLSSSGIMVVLTCRDVTRGLEAVEKLKNSNHENVVFHQLDVTDPITTMSSLADFIKARFGKLDILVNNAGVAGFSVDADRFKAMISDIGEDSEEVVKIYEKPEAQELMSETYELAEECLKINYYGVKSVTEVLLPLLQLSDSPRIVNVSSSTGSLKYVSNETALEILGDGDALTEERIDMVVNMLLKDFKENLIETNGWPSFGAAYTTSKACLNAYTRVLAKKIPKFQVNCVCPGLVKTEMNYGIGNYTADEGAKHVVRIALFPDDGPSGFFYDCSELSAF

SEQ ID NO: 94 - protein, 343 aa, Z. mays
MSTGGRKMRTACVTGGNGYIASALIKVLLEKGYAVKTTVRNPDDMEKNSHLKDLQALGSLEVFRADLDEDGSFDDAVAGCDYAFLVAAPVNLHTKNPEEEMIEPAVRGTLNVMRSCVKAGTVRRVVLTSSAAAVTTRPQLQGDGHVLDEESWSDVEYLRAHKPAGPWGYPVSKVLLEKEASRFAEEHGIGLVTVCPGLTVGAAPAPTARTSVPNCLSLLSGDEAAFAVLDAIESATGCLPLVHVDDVCRAELFAAEEGAAARRYVCCGLNTTVAELARFLADKYPQYGVKTNLLSGERLEKPRVCLSSAKLVKEGFEFRYRTLDDIYDDMVEYGKALGILPDL

SEQ ID NO: 95 - protein, 340 aa, A. thaliana
MDQTLTHTGSKKACVIGGTGNLASILIKHLLQSGYKVNTTVRDPENEKKIAHLRKLQELGDLKIFKADLTDEDSFESSFSGCEYIFHVATPINFKSEDPEKDMIKPAIQGVINVLKSCLKSKSVKRVIYTSSAAAVSINNLSGTGIVMNEENWTDVEFLTEEKPFNWGYPISKVLAEKTAWEFAKENKINLVTVIPALIAGNSLLSDPPSSLSLSMSFITGKEMHVTGLKEMQKLSGSISFVHVDDLARAHLFLAEKETASGRYICCAYNTSVPEIADFLIQRYPKYNVLSEFEEGLSIPKLTLSSQKLINEGFRFEYGINEMYDQMIEYFESKGLIKAK

SEQ ID NO: 96 - protein, 348 aa, P. somniferum
MHGQKNISERYQKFKEMEGTGKIVCVTGGAGYLASWLIMRLLERGYSVRTTVRSDPKFREDVSHLKALPEATEKLQIFEADLENPESFDDAINGCVGVFLVAQGMNFAEEYTLEKIIKTCVEGTLRILQSCLKSKTVKKVVYTSSADAAMMISNLKAVKEIDETIWSEVDNFISKPEQVIPGLPSYVVSKVLTERACLKFSEEHGLDVVTILPPLVVGPFITPHPPPSVSIALSIISGDVSMMLGVRLENAVHIDDVALAHIFVFECEKAKGRHICSSVDFPMHDLPKFISENYPEFNVPTDLLKDIEEQEPVHLSSDKLLSMGFQFKYDFAEIFGDAIRCAKEKGFL

SEQ ID NO: 97 - protein, 360 aa, A. thaliana
MVREEEEDDNNGGGGERKLPVADETVPSLLDGTGLVCVTGGTGFVASWLIMRLLQRGYSVRATVRTNPEGNKKDISYLTELPFASERLQIFTADLNEPESFKPAIEGCKAVFHVAHPMDPNSNETEETVTKRTVQGLMGILKSCLDAKTVKRFFYTSSAVTVFYSGKNGGGGGEVDESVWSDVEVFRNQKEKRVSSSYVVSKMAAETAALEFGGKNGLEVVTLVIPLVVGPFISPSLPSSVFISLAMLFGNYKEKYLFDTYNMVHIDDVARAMILLLEKPVAKGRYICSSVEMKIDEVFEFLSTKFPQFQLPSIDLKNYKVEKRMSLSSKKLRSEGFEFKYGAEEIFGGAIRSCQARGFL

SEQ ID NO: 98 - protein, 323 aa, Homo sapiens
MDPKYQRVELNDGHFMPVLGFGTYAPPEVPRNRAVEVTKLAIEAGFRHIDSAYLYNNEEQVGLAIRSKIADGSVKREDIFYTSKLWCTFFQPQMVQPALESSLKKLQLDYVDLYLLHFPMALKPGETPLPKDENGKVIFDTVDLSATWEVMEKCKDAGLAKSIGVSNFNCRQLEMILNKPGLKYKPVCNQVECHPYLNQSKLLDFCKSKDIVLVAHSALGTQRHKLWVDPNSPVLLEDPVLCALAKKHKRTPALIALRYQLQRGVVVLAKSYNEQRIRENIQVFEFQLTSEDMKVLDGLNRNYRYVVMDFLMDHPDYPFSDEY

SEQ ID NO: 99 - protein, 323 aa, Mus musculus
MDSKQQTVRLSDGHFIPILGFGTYAPQEVPKSKATEATKIAIDAGFRHIDSASMYQNEKEVGLAIRSKIADGTVKREDIFYTSKVWCTFHRPELVRVCLEQSLKQLQLDYVDLYLIHFPMAMKPGENYLPKDENGKLIYDAVDICDTWEAMEKCKDAGLAKSIGVSNFNRRQLEKILKKPGLKYKPVCNQVECHPYLNQGKLLDFCRSKDIVLVAYSALGSHREKQWVDQSSPVLLDNPVLGSMAKKYNRTPALIALRYQLQRGVVVLAKSFSEKRIKENMQVFEFQLTSEDMKVLDDLNKNIRYISGSSFKDHPDFPFWDEY

SEQ ID NO: 100 - protein, 317 aa, S. lycopersicum
MAEATEMPYIELNTGFSIPAVGLGTWQSDPGVVGKAVETAIKMGYRHIDCAQIYKNEKEIGEVLSRLFKDGVVKRRELFITSKLWNTNHAPEDVPVALDKTLQDLQLEYVDLYLIHWPVSMKPGSVDFKPENLMPTNIPRIWEAMEKVYDSGKARVIGVSNFSTKKLEDLLQVARTPPAVNQVECHPSWQQAKLRELCKSNNVHLSAYSPLGSPGTTWLKSDVLKQPAVISVAEKLGKTPAQVCLRWGIQMGQSVLPKSTHEARIKENLDVLNWSIPDDLLAKFSEIPQARLLKGASFAHETHGQYRTLEELWDGEI

SEQ ID NO: 101 - protein, 331 aa, S. lycopersicum
MTMNLIKQMLVPNVNLNSGHKMPLIGMGTAPSLPEHDQLVSTLIDAIEIGYRHFDTAAVYGSEEALGQAVVEAIQRGLIKSREQVFITSKLWCTETHRHLVLPALKRTLGRLKMDYLDLYLIHLPVTMKKKVNSKDDEMRVDKEDIIPFDMRGTWEAMEECCRLGLAKSIGVSNFTCTKISQILHYATILPAVNQVEMHVAWRQEKMLEFCKEKGIHVSAWSPLGANGLTPWGIHSVMESPVLKDIAIHKRKSVAQVALRWVYEQGASVIVKSFNKERMKENLQILDWELSNEEIAQIQEIPPCTGFNVDMVLVHPNGPYKSANQFWDGEI

SEQ ID NO: 102 - protein, 312 aa, M. truncatula
MGSVEIPTKVLTNTSSQLKMPVVGMGSAPDFTCKKDTKDAIIEAIKQGYRHFDTAAAYGSEQALGEALKEAIELGLVTRQDLFVTSKLWVTENHPHLVIPALQKSLKTLQLDYLDLYLIHWPLSSQPGKFTFPIDVADLLPFDVKGVWESMEEGLKLGLTKAIGVSNFSVKKLENLLSVATILPAVNQVEMNLAWQQKKLREFCNANGIVLTAFSPLRKGASRGPNEVMENDMLKEIADAHGKSVAQISLRWLYEQGVTFVPKSYDKERMNQNLCIFDWSLTKEDHEKIDQIKQNRLIPGPTKPGLNDLYDD

SEQ ID NO: 103 - protein, 321 aa, P. somniferum
MESNGVPMITLSSGIRMPALGMGTAETMVKGTEREKLAFLKAIEVGYRHFDTAAAYQTEECLGEAIAEALQLGLIKSRDELFITSKLWCADAHADLVLPALQNSLRNLKLDYLDLYLIHHPVSLKPGKFVNEIPKDHILPMDYKSVWAAMEECQTLGFTRAIGVCNFSCKRLQELMETANSPPVVNQVEMSPTLHQKNLREYCKANNIMITAHSVLGAVGAAWGTNAVMHSKVLHQIAVARGKSVAQVSMRWVYQQGASLVVKSFNEARMKENLKIFDWELTAEDMEKISEIPQSRTSSAAFLLSPTGPFKTEEEFWDEKD

SEQ ID NO: 104 - protein, 320 aa, A. thaliana
MSALTFPIGSVHHLMPVLALGTAASPPPEPIVLKRTVLEAIKLGYRHFDTSPRYQTEEPLGEALAEAVSLGLIQSRSELFVTSKLWCADAHGGLVVPAIQRSLETLKLDYLDLYLIHWPVSSKPGKYKFPIEEDDFLPMDYETVWSEMEECQRLGVAKCIGVSNFSCKKLQHILSIAKIPPSVNQVEMSPVWQQRKLRELCKSKGIVVTAYSVLGSRGAFWGTHKIMESDVLKEIAEAKGKTVAQVSMRWAYEEGVSMVVKSFRKDRLEENLKIFDWSLTEEEKQRISTEISQSRIVDGEVYISEKGPIKSVTEMWDGEI

SEQ ID NO: 105 - protein, 259 aa, D. lanata
MSSKPRLEGKVAIITGAASGIGEETARLFVEHGASVVVADVQDELGRQVVASVNSDDKISYYHCDVRDEKQVAATVRYAVEKYGRLDIMLSNAGVFGALMTNVIDLDMVDFENVLATNVRGVANTIKHAARAMVEGKVKGSIICTASVSASLGGMGPPAYTASKHAVLGLVKGACAELGVHGIRVNSVAPYGVATPMPCSAYGMTPSQMEEANNSRANLKGVVLKAKHVAEAALFLASDESAYVSGQNLAVDGGFTVVR

SEQ ID NO: 106 - DNA, 33 bp, synthetic construct
  misc_feature 1..33: note = GAME25 silencing construct for S. pennellii forward primer
  source 1..33: mol_type = other DNA
gcggccgcattgtcactctattgtgttggcgtg

SEQ ID NO: 107 - DNA, 36 bp, synthetic construct
  misc_feature 1..36: note = GAME25 silencing construct for S. pennellii reverse primer
  source 1..36: mol_type = other DNA
ggcgcgcctaaatttatatcttttcaagtcacaatg